European Patent Specification EP 3 557 996 B1, published January 10, 2024. Title: NOVEL INSECT INHIBITORY PROTEINS. Applicant: Monsanto Technology LLC. The sequence listing filed with the application follows.

SEQUENCE LISTING (99 sequences)

SEQ ID NO: 1 - DNA, 891 bp, Artificial
  Nucleic acid sequence obtained from the Lysinibacillus sphaericus species AG0067H07 encoding a TIC6280 pesticidal protein with a Histidine tag operably linked to the 3' end, TIC6280-His.
atgtcaaatcaagatttacagatggaaagctggttaacattaaatgatgtttcccttcatcaaaatattcaaacaccactttctttcgaccttacttcctctttacaagatgctgcacctgtccaagatactataagtggaggtttaattattggtaacacacaaaacgaagctatcgatgccaataataatgtaaaaaatgcactgcaaacatacggtcgttttagtaatgaggtcaaagaatctgctcaagtaagtccgattgttggattaacaactatacttgatattgcaagaatagtttccaattacaacccggctttgcccactgatcaagaaaatgatgaaactaaaaaagcaagagttattgcatacaaccaatatattacgaaggtgttgcaaaatcctttaatgcacttaaaaagcaactatgaaaaaaaatacacaaaacgaacttctaactggaagacagctattgatgaaatcagtaatttatatgatggcatcacagaaaaagataaagagaaaattaaaaatagtttacaagctttagcagaagctgcttcttcaagatcaaatcaagccaatacagaaaatatatttgctcaaaatgttattgtgtgcaatgatgaagaaattgaattttgtatttattcaagttcagttacaatgctttatagtggtggtaaaaataccgtaagacaggttgatttcactctaaacgaaacccacattagatttacaaaagagttatggagtagatactctgataaagttttagataaacacttagcgttgatagatgattggctacttggaattagtactcctaatagtgataaaactactctcgcttgctttgttcaccaccatcacgctcaccatcactga

SEQ ID NO: 2 - protein, 296 aa, Artificial
  Amino acid sequence of the TIC6280-His protein.
MSNQDLQMESWLTLNDVSLHQNIQTPLSFDLTSSLQDAAPVQDTISGGLIIGNTQNEAIDANNNVKNALQTYGRFSNEVKESAQVSPIVGLTTILDIARIVSNYNPALPTDQENDETKKARVIAYNQYITKVLQNPLMHLKSNYEKKYTKRTSNWKTAIDEISNLYDGITEKDKEKIKNSLQALAEAASSRSNQANTENIFAQNVIVCNDEEIEFCIYSSSVTMLYSGGKNTVRQVDFTLNETHIRFTKELWSRYSDKVLDKHLALIDDWLLGISTPNSDKTTLACFVHHHHAHHH

SEQ ID NO: 3 - DNA, 891 bp, Artificial
  Nucleic acid sequence obtained from the Lysinibacillus sphaericus species AG0067H03 encoding a TIC6281 pesticidal protein with a Histidine tag operably linked to the 3' end, TIC6281-His.
atgtcaaatcaagatttacagatggaaagctggttaacattaaatgatgtttcccttcatcaaaatattcaaacaccactttctttcgaccttacttcctctttacaagatgctgcacctgtccaagatactataagtggaggtttaattattggtaacacacaaaacgaagctatcgatgccagtaataatgtaaaaaatgcactgcaaacatacggtcgttttagtaatgaggtcaaagaatctgctcaagtaagtccgattgttggattaacaactatacttgatattgcaagaatagtttccaattacaacccggctttgcccactgatcaagaaaatgatgaaactaaaaaagcaagagttattgcatacaaccaatatattacgaaggtgttgcaaaatcctttaatgcacttaaaaagcaactatgaaaaaaaatacacaaaacgaacttctaactggaagacagctattgatgaaatcagtaatttatatgatggcatcacagaaaaagataaagagaaaattaaaaatagtttacaagctttagcagaagctgcttcttcaagatcaaatcaagccaatacagaaaatatatttgctcaaaatgttattgtgtgcaataatgaagaaattgaattttgtatttattcaagttcagttacaatgctttatagtggtggtaaaaataccgtaagacaggttgatttcactctaaacgaaacccacattagatttacaaaagagttatggagtagatactctgataaagttttagataaacacttagcgttgatagatgattggctacttggaattagtactcctaatagtgataaaactactctcgcttgctttgttcaccaccatcacgctcaccatcactga

SEQ ID NO: 4 - protein, 296 aa, Artificial
  Amino acid sequence of the TIC6281-His protein.
MSNQDLQMESWLTLNDVSLHQNIQTPLSFDLTSSLQDAAPVQDTISGGLIIGNTQNEAIDASNNVKNALQTYGRFSNEVKESAQVSPIVGLTTILDIARIVSNYNPALPTDQENDETKKARVIAYNQYITKVLQNPLMHLKSNYEKKYTKRTSNWKTAIDEISNLYDGITEKDKEKIKNSLQALAEAASSRSNQANTENIFAQNVIVCNNEEIEFCIYSSSVTMLYSGGKNTVRQVDFTLNETHIRFTKELWSRYSDKVLDKHLALIDDWLLGISTPNSDKTTLACFVHHHHAHHH

SEQ ID NO: 5 - DNA, 891 bp, Artificial
  Nucleic acid sequence obtained from the Lysinibacillus sphaericus species AG0069H08 encoding a TIC6282 pesticidal protein with a Histidine tag operably linked to the 3' end, TIC6282-His.
atgtcaaatcaagatttacagatggaaagctggttaacagtaaatgatgtttcccttcatcaaaatattcaaacaccactttctttcgaccttacatcctctttacaagatgctgcacctgtccaagatactataagtggaggtttaattattggtaacacacaaaacgaagctatcgatgccaataataatgtaaaaaatgcactgcaaacatacggtcgttttagtaatgaggtcaaagaatctgctcaagtaagtccgattgttggattaacaactatacttgatattgcaagaatagtttccaattacaacccggctttgcccactgatcaagaaaatgatgaaactaaaaaagcaagagttattgcatacaaccaatatattacgaaggtgttgcaaaatcctttaatgcacttaaaaagcaactatgaaaaaaaatacacaaaacgaacttctaactggaagacagctattgaggaaatcagtaatttatatgatggcatcacagaaaaagataaagagaaaattaaaaatagtttacaagctttagcagaagctgcctcttcaagatcaaatcaagccaatacagaaaatatatttgctcaaaatgttattgtgtgcaatgatgaagaaattgaattttgtatttattcaagttcagttacaatgctttatagtggtggtaaaaataccgtaagacaggttgatttcactctaaacgaaacccacattagatttacaaaagagttatggagtagatactctgataaagttttagataaacacttagcgttgatagatgattggctacttggaattagtactcctaatagtgataaaactactctcgcttgctttgttcaccaccatcacgctcaccatcactga

SEQ ID NO: 6 - protein, 296 aa, Artificial
  Amino acid sequence of the TIC6282-His protein.
MSNQDLQMESWLTVNDVSLHQNIQTPLSFDLTSSLQDAAPVQDTISGGLIIGNTQNEAIDANNNVKNALQTYGRFSNEVKESAQVSPIVGLTTILDIARIVSNYNPALPTDQENDETKKARVIAYNQYITKVLQNPLMHLKSNYEKKYTKRTSNWKTAIEEISNLYDGITEKDKEKIKNSLQALAEAASSRSNQANTENIFAQNVIVCNDEEIEFCIYSSSVTMLYSGGKNTVRQVDFTLNETHIRFTKELWSRYSDKVLDKHLALIDDWLLGISTPNSDKTTLACFVHHHHAHHH

SEQ ID NO: 7 - DNA, 891 bp, Artificial
  Nucleic acid sequence obtained from the Lysinibacillus sphaericus species AG0025E04 encoding a TIC6283 pesticidal protein with a Histidine tag operably linked to the 3' end, TIC6283-His
atgtcaaatcaagatttacagatggaaagctggttaacagtaaatgatgtttcccttcatcaaaatattcaaacaccactttctttcgaccttacatcctctttacaagatgttgcacctgtccaagatactataagtggaggtttaattattggtaacacacaaaacgaagctatcgatgccaataataatgtaaaaaatgcactgcaaacatacggtcgttttagtaatgaggtcaaagaatctgctcaagtaagtccgattgttggattaacaactatacttgatattgcaagaatagtttccaattacaacccggctttgcccactgatcaagaaaatgatgaaactaaaaaagcaagagttattgcatacaaccaatatattacgaaggtgttgcaaaatcctttaatgcacttaaaaagcaactatgaaaaaaattacacaaaacgaacttctaactggaagacagctattgaggaaatcagtaatttatatgatggcatcacagaaaaagataaagagaaaattaaaaatagtttacaagctttagcagaagctgcctcttcaagatcaaatcaagccaatacagaaaatatatttgctcaaaatgttattgtgtgcaatgatgaagaaattgaattttgtatttattcaagttcagttacaatgctttatagtggtggtaaaaataccgtaagacaggttgatttcactctaaacgaaacccacattagatttacaaaagagttatggagtagatactctgataaagttttagataaacacttagcgttgatagatgattggctacttggaattagtactcctaatagtgataaaactactctcgcttgctttgttcaccaccatcacgctcaccatcactga

SEQ ID NO: 8 - protein, 296 aa, Artificial
  Amino acid sequence of the TIC6283-His protein.
MSNQDLQMESWLTVNDVSLHQNIQTPLSFDLTSSLQDVAPVQDTISGGLIIGNTQNEAIDANNNVKNALQTYGRFSNEVKESAQVSPIVGLTTILDIARIVSNYNPALPTDQENDETKKARVIAYNQYITKVLQNPLMHLKSNYEKNYTKRTSNWKTAIEEISNLYDGITEKDKEKIKNSLQALAEAASSRSNQANTENIFAQNVIVCNDEEIEFCIYSSSVTMLYSGGKNTVRQVDFTLNETHIRFTKELWSRYSDKVLDKHLALIDDWLLGISTPNSDKTTLACFVHHHHAHHH

SEQ ID NO: 9 - DNA, 849 bp, Artificial
  Nucleic acid sequence obtained from the Lysinibacillus sphaericus species EGBS0420 encoding a TIC7016 pesticidal protein with a Histidine tag operably linked to the 3' end, TIC7016-His.
atgacaaatcttgacttaaaaatggaaagttggttagcactaaatgatatttctctacatcaaaatttagagcctgttgctattaaactcgcaacatcagatcaaacagttgtcagtcaaggaatctttgtagggaatcagttgtcggaggctagaattgctgacaatcaggttcagcaggcacttcaaagctttggacgctatagtactgctgtaaaagaagctgctaaagtagctccaacaactggtttaacaactatccttgacattgctagaatcgtttctaatttcaatccggcattaccaaacgataaaaataatgtacctgcctatgaaaaatatgtttcaaaaatattacaaaacccacttatccatttattaaatagcagtgtaaaatccttcaaacgtacgacttctgattggaatgaagcaattgaccaaattgccaatttatataatggcatttcggcagctgacaaaggaaaaattgtagaaagcttaaaagcattagcaaaatccgcctcctcttctagctctgaaaaacaaacggaaaaactatttactcaaagtacgattaactgtgaggaaaatatagatatttatatttactctagctctgtcacaatggaggagcacaacggtaagcacaatgtaaagcaggttgaatttgaaatacaagaaacacaattaagatttacaaaagaattgtggagtttatactctgatgctgtgttagctaaacatctagctctaatggatgattggctaaatggcattgatacaaaagcagacaatcgtttatccactcttacatgcttagttcaccaccatcacgctcaccatcactga

SEQ ID NO: 10 - protein, 282 aa, Artificial
  Amino acid sequence of the TIC7016-His protein.
MTNLDLKMESWLALNDISLHQNLEPVAIKLATSDQTVVSQGIFVGNQLSEARIADNQVQQALQSFGRYSTAVKEAAKVAPTTGLTTILDIARIVSNFNPALPNDKNNVPAYEKYVSKILQNPLIHLLNSSVKSFKRTTSDWNEAIDQIANLYNGISAADKGKIVESLKALAKSASSSSSEKQTEKLFTQSTINCEENIDIYIYSSSVTMEEHNGKHNVKQVEFEIQETQLRFTKELWSLYSDAVLAKHLALMDDWLNGIDTKADNRLSTLTCLVHHHHAHHH

SEQ ID NO: 11 - DNA, 849 bp, Artificial
  Nucleic acid sequence obtained from the Lysinibacillus sphaericus species EGBS1094 encoding a TIC7017 pesticidal protein with a Histidine tag operably linked to the 3' end, TIC7017-His.
atgacaaatcttgacttaaaaatggaaagttggttagcactaaatgatatttctctacatcaaaatttagagcctgttgctattaaactcgcaacatcagatcaaacagttgtcagtcaaggaatctttgttgggaatcagctgtcggaggctagaattgctgacaaccaagttcagcaagcacttcaaagctttggacgctatagtgctgctgtaaaagaagctgctaaaatagctccaacaactggattaacaactatccttgacattgctagaattgtttctaatttcaatcctgcattaccaaacgataaaaataatgtacctgcctatgaaaaatatgtttcaaaaatattacaaaacccacttatccatttattaaatagcagtgtaaaatcctttaaacgtacgacttccgattggaatgaagcaattgaccaaattgccaatttatataatggcatttcggcagctgacaaaggaaaaattgtagaaagcttaaaagcattagcaaaatccgcctcttcttctagctctgaaaaacaaacggaaaaactatttactcaaagtacgattaactgtgaggaaaatattgatatttatatttactctagctctgtcacaatggaggagcacagcggtaagcataatgtaaagcaggttgaatttgaaatacaagaaacacaattaagatttacaaaagaattgtggagtttatactcagatgctgtgttagctaaacatctagcattaatggatgattggctgaatggcattgatacaaaagcagacaaccgtttatccactcttacatgcttagttcaccaccatcacgctcaccatcactga

SEQ ID NO: 12 - protein, 282 aa, Artificial
  Amino acid sequence of the TIC7017-His protein.
MTNLDLKMESWLALNDISLHQNLEPVAIKLATSDQTVVSQGIFVGNQLSEARIADNQVQQALQSFGRYSAAVKEAAKIAPTTGLTTILDIARIVSNFNPALPNDKNNVPAYEKYVSKILQNPLIHLLNSSVKSFKRTTSDWNEAIDQIANLYNGISAADKGKIVESLKALAKSASSSSSEKQTEKLFTQSTINCEENIDIYIYSSSVTMEEHSGKHNVKQVEFEIQETQLRFTKELWSLYSDAVLAKHLALMDDWLNGIDTKADNRLSTLTCLVHHHHAHHH

SEQ ID NO: 13 - DNA, 849 bp, Artificial
  Nucleic acid sequence obtained from the Lysinibacillus sphaericus species AG0025E04 encoding a TIC7107 pesticidal protein with a Histidine tag operably linked to the 3' end, TIC7107-His.
atgacaaatcttgacttaaaaatggaaagctggttagcactaaatgatatttctctgcatcaaaatttagagcctgttgctattaaacttgctccatcagatcaaacagttgtcagtcaaggaatctttgttgggagtcagctgtcggaggctagaatcgctgacaatcaagttcagcaagcacttcaaaactttggacgctatagttctgcggtaaaagaagctgctaaagtagctccaacaactggattaacaactattcttgacattgctagaattgtctctaattttaatccagcattaccaaacgataaaaataatgttcctgcttatgaaaaatatgtgtcaaaaattttacaaaacccacttatccatttattaaatagcagtctaaaatcctttaaacgtaggacttccgattggaatgaagtaattgaccaaatcgccaatttatataatggcatttcggcagttgataaaggaaaaatcgtagaaagcttaaaagcattagcaaattccgcctcttcttctagctcagaaaaacaaactgaaaaactatttactcaaagcacgattaactgtgaggaaaatattgatatttatatttactctagctctgttacaatggaggagcacaatgggaagcataatgtaaaacaagttgaatttgaaatacaagaaacacaattaagatttacaaaagaattgtggagtttatactcagatgctgtgttagcaaaacatctagctttaatggatgattggctcaatggcattgatacaaaagctgacaatcgtttatccactcttacatgcttagttcaccaccatcacgctcaccatcactga

SEQ ID NO: 14 - DNA, 849 bp, Artificial
  Nucleic acid sequence obtained from the Lysinibacillus sphaericus species AG0067H01 encoding a TIC7108 pesticidal protein with a Histidine tag operably linked to the 3' end, TIC7108-His.
atgacaaatcttgacttaaaaatggaaagctggttagcactaaatgatatttctctgcatcaaaatttagagcctgttgctattaaacttgcaccatcagatcaaacagttgtcagtcaaggaatctttgttgggagtcagctgtcggaggctagaatcgctgacaatcaagttcagcaagcacttcaaaactttggacgctatagttctgcagtaaaagaagctgctaaagtagctccaacaactggattaacaactattcttgatattgctagaattgtttctaattttaatccagcattaccaaacgataaaaataatgttcctgcttatgaaaaatatgtgtcaaaaattttacaaaacccacttatccatttattaaatagcagtctaaaatcctttaaacgtaggacttccgattggaatgaagtaattgaccaaatcgccaatttatataatggcatttcggcagttgataaaggaaaaatcgtagaaagcttaaaagcattagcaaattccgcctcttcttctagctcagaaaaacaaattgaaaaactatttactcaaagcacgattaactgtgaggaaaatattgatatttatatttactctagctctgttacaatggaggagcacaatgggaagcataatgtaaagcaagttgaatttgaaatacaagaaacacaattaagatttacaaaagaattgtggagtttatactcagatgctgtgttagcaaaacatctagctttaatggatgattggctcaatggcattgatacaaaagctgacaatcgtttatccactcttacatgcttagttcaccaccatcacgctcaccatcactga

SEQ ID NO: 15 - protein, 282 aa, Artificial
  Amino acid sequence of the TIC7108-His protein.
MTNLDLKMESWLALNDISLHQNLEPVAIKLAPSDQTVVSQGIFVGSQLSEARIADNQVQQALQNFGRYSSAVKEAAKVAPTTGLTTILDIARIVSNFNPALPNDKNNVPAYEKYVSKILQNPLIHLLNSSLKSFKRRTSDWNEVIDQIANLYNGISAVDKGKIVESLKALANSASSSSSEKQIEKLFTQSTINCEENIDIYIYSSSVTMEEHNGKHNVKQVEFEIQETQLRFTKELWSLYSDAVLAKHLALMDDWLNGIDTKADNRLSTLTCLVHHHHAHHH

SEQ ID NO: 16 - DNA, 849 bp, Artificial
  Nucleic acid sequence obtained from the Lysinibacillus sphaericus species AG0067H03 encoding a TIC7109 pesticidal protein with a Histidine tag operably linked to the 3' end, TIC7109-His.
atgacaaatcttgacttaaaaatggaaagctggttagcactaaatgatatttctctgcatcaaaatttagagcctgttgctattaaacttgcaccatcagatcaaacagttgtcagtcaaggaatctttgttgggagtcagctgtcggaggctagaatcgctgacaatcaagttcagcaagcacttcaaaactttggacgctatagttctgcagtaaaagaagctgctaaagtagctccaacaactggattaacaactattcttgatattgctagaattgtttctaattttaatccagcattaccaaacgataaaaataatgttcctgcttatgaaaaatatgtgtcaaaaattttacaaaacccacttatccatttattaaatagcagtctaaaatcctttaaacgtaggacttccgattggaatgaagtaattgaccaaatcgccaatttatataatggcatttcggcagttgataaaggaaaaatcgtagaaagcttaaaagcattagcaaattccgcctcttcttctagctcagaaaaacaaactgaaaaactatttactcaaagcacgattaactgtgaggaaaatattgatatttatatttactctagctctgttacaatggaggagcacaatgggaagcataatgtaaagcaagttgaatttgaaatacaagaaacacaattaagatttacaaaagaattgtggagtttatactcagatgctgtgttagcaaaacatctagctttaatggatgattggctcaatggcattgatacaaaagctgacaatcgtttatccactcttacatgcttagttcaccaccatcacgctcaccatcactga

SEQ ID NO: 17 - DNA, 849 bp, Artificial
  Nucleic acid sequence obtained from the Lysinibacillus sphaericus species AG0067H07 encoding a TIC7110 pesticidal protein with a Histidine tag operably linked to the 3' end, TIC7110-His.
atgacaaatcttgacttaaaaatggaaagctggttagcactaaatgatatttctctgcatcaaaatttagagcctgttgctattaaacttgcaccatcagatcaaacagttgtcagtcaaggaatctttgttgggagtcagctgtcggaggctagaatcgctgacaatcaagttcagcaagcacttcaaaactttggacgctatagttctgcagtaaaagaagctgctaaagtagctccaacaactggattaacaactattcttgatattgctagaattgtttctaattttaatccagcattaccaaacgataaaaataatgttcctgcttatgaaaaatatgtgtcaaaaattttacaaaacccacttatccatttattaaatagcagtctaaaatcctttaaacgtaggacttccgattggaatgaagtaattgaccaaatcgccaatttatataatggcatttcggcagttgataaaggaaaaatcgtagaaagcttaaaagcattagcaaattccgcctcttcttctagctcagaaaaacaaactgaaaaactatttactcaaagcacgattaactgtgaggaaaatattgatatttatatttactctagctctgttacaatggaggagcacaatgggaagcataatgtaaagcaagttgaatttgaaatacaagaaactcaattaagatttacaaaagaattgtggagtttatactcagatgctgtgttagcaaaacatctagctttaatggatgattggctcaatggcattgatacaaaagctgacaatcgtttatccactcttacatgcttagttcaccaccatcacgctcaccatcactga

SEQ ID NO: 18 - protein, 282 aa, Artificial
  Amino acid sequence of the TIC7110-His protein.
MTNLDLKMESWLALNDISLHQNLEPVAIKLAPSDQTVVSQGIFVGSQLSEARIADNQVQQALQNFGRYSSAVKEAAKVAPTTGLTTILDIARIVSNFNPALPNDKNNVPAYEKYVSKILQNPLIHLLNSSLKSFKRRTSDWNEVIDQIANLYNGISAVDKGKIVESLKALANSASSSSSEKQTEKLFTQSTINCEENIDIYIYSSSVTMEEHNGKHNVKQVEFEIQETQLRFTKELWSLYSDAVLAKHLALMDDWLNGIDTKADNRLSTLTCLVHHHHAHHH

SEQ ID NO: 19 - DNA, 849 bp, Artificial
  Nucleic acid sequence obtained from the Lysinibacillus sphaericus species AG0069H08 encoding a TIC7111 pesticidal protein with a Histidine tag operably linked to the 3' end, TIC7111-His.
atgacaaatcttgacttaaaaatggaaagctggttagcactaaatgatatttctctgcatcaaaatttagagcctgttgctattaaacttgcaccatcagatcaaacagttgtcagtcaaggaatctttgttgggagtcagctgtcggaggctagaatcgctgacaatcaagttcagcaagcacttcaaaactttggacgctatagttctgcagtaaaagaagctgctaaagtagctccaacaactggattaacaactattcttgacattgctagaattgtctctaattttaatccagcattaccaaacgataaaaataatgttcctgcttatgaaaaatatgtgtcaaaaattttacaaaacccacttatccatttattaaatagcagtctaaaatcctttaaacgtaggacttccgattggaatgaagtaattgaccaaatcgccaatttatataatggcatttcggcagttgataaaggaaaaatcgtagaaagcttaaaagcattagcaaattccgcctcttcttctagctcagaaaaacaaactgaaaaactatttactcaaagcacgattaactgtgaggaaaatattgatatttatatttactctagctctgttacaatggaggagcacaatgggaagcataatgtaaagcaagttgaatttgaaatacaagaaacacaattaagatttacaaaagaattgtggagtttatactcagatgctgtgttagcaaaacatctagctttaatggatgattggctcaatggcattgatacaaaagctgacaatcgtttatccactcttacatgcttagttcaccaccatcacgctcaccatcactga

SEQ ID NO: 20 - DNA, 852 bp, Artificial
  Nucleic acid sequence obtained from the Lysinibacillus sphaericus species AG0122F12 encoding a TIC7589 pesticidal protein with a Histidine tag operably linked to the 3' end, TIC7589-His.
atgacaaatcttgatttaaaaatggaaagttggttggctgtaaatgatgtttctcaccaccagaatcttcaacaaccatattctgagatttcatcaacatctgaagaagtacttgtaagtcaaggattatttgtaggtgataaattggaaaacgcaataagtgcagataccaatgtccaacaagcacttcaaacatacggtcgttatagcgacgcagtaaaagaagcaactaaacttgcaccaacaaccggcttaacaacgttacttgatatttcacgaattgtttctggctttaatccagatttacctaatgatcctaaaaatgtccaagcatacaatcaatacattacaacaatattgaaaaatcctctttttcatttactaaaatctgaaagagtaaagtttacgagagctacatcagactggaatgaagcaattgataaaattgcggatctttatgatggtatacctacatctgataaaagtaagattgtaaaaagcttaaagacattagcagaagccgcctcttcttataccgaaaccaaccaaacagattatttatttacccaaagtacagtaaattgcagtgacaatattgatgtttatatttactcaagtacagtgacattgaaagaaaaaagtgggaaacatcacgtaaaagaatctacccttgatataggctgcgtacaattaagatttacaaaagagttatggagtgtatactctgatgaagtcttaaaaagacatttagcgttgatgactgattggttaaatgccatgaattcgaaaccaggaactaaacaatcgaaactcacttgcttagttcaccaccatcacgctcaccatcactga

SEQ ID NO: 21 - protein, 283 aa, Artificial
  Amino acid sequence of the TIC7589-His protein.
MTNLDLKMESWLAVNDVSHHQNLQQPYSEISSTSEEVLVSQGLFVGDKLENAISADTNVQQALQTYGRYSDAVKEATKLAPTTGLTTLLDISRIVSGFNPDLPNDPKNVQAYNQYITTILKNPLFHLLKSERVKFTRATSDWNEAIDKIADLYDGIPTSDKSKIVKSLKTLAEAASSYTETNQTDYLFTQSTVNCSDNIDVYIYSSTVTLKEKSGKHHVKESTLDIGCVQLRFTKELWSVYSDEVLKRHLALMTDWLNAMNSKPGTKQSKLTCLVHHHHAHHH

SEQ ID NO: 22 - DNA, 867 bp, Lysinibacillus sphaericus
  misc_feature (1)..(867): Nucleic acid sequence obtained from the Lysinibacillus sphaericus species AG0067H07 encoding a TIC6280 pesticidal protein.
atgtcaaatcaagatttacagatggaaagctggttaacattaaatgatgtttcccttcatcaaaatattcaaacaccactttctttcgaccttacttcctctttacaagatgctgcacctgtccaagatactataagtggaggtttaattattggtaacacacaaaacgaagctatcgatgccaataataatgtaaaaaatgcactgcaaacatacggtcgttttagtaatgaggtcaaagaatctgctcaagtaagtccgattgttggattaacaactatacttgatattgcaagaatagtttccaattacaacccggctttgcccactgatcaagaaaatgatgaaactaaaaaagcaagagttattgcatacaaccaatatattacgaaggtgttgcaaaatcctttaatgcacttaaaaagcaactatgaaaaaaaatacacaaaacgaacttctaactggaagacagctattgatgaaatcagtaatttatatgatggcatcacagaaaaagataaagagaaaattaaaaatagtttacaagctttagcagaagctgcttcttcaagatcaaatcaagccaatacagaaaatatatttgctcaaaatgttattgtgtgcaatgatgaagaaattgaattttgtatttattcaagttcagttacaatgctttatagtggtggtaaaaataccgtaagacaggttgatttcactctaaacgaaacccacattagatttacaaaagagttatggagtagatactctgataaagttttagataaacacttagcgttgatagatgattggctacttggaattagtactcctaatagtgataaaactactctcgcttgctttgtttaa

SEQ ID NO: 23 - protein, 288 aa, Lysinibacillus sphaericus
  MISC_FEATURE (1)..(288): Amino acid sequence of the TIC6280 protein.
MSNQDLQMESWLTLNDVSLHQNIQTPLSFDLTSSLQDAAPVQDTISGGLIIGNTQNEAIDANNNVKNALQTYGRFSNEVKESAQVSPIVGLTTILDIARIVSNYNPALPTDQENDETKKARVIAYNQYITKVLQNPLMHLKSNYEKKYTKRTSNWKTAIDEISNLYDGITEKDKEKIKNSLQALAEAASSRSNQANTENIFAQNVIVCNDEEIEFCIYSSSVTMLYSGGKNTVRQVDFTLNETHIRFTKELWSRYSDKVLDKHLALIDDWLLGISTPNSDKTTLACFV

SEQ ID NO: 24 - DNA, 867 bp, Lysinibacillus sphaericus
  misc_feature (1)..(867): Nucleic acid sequence obtained from the Lysinibacillus sphaericus species AG0067H03 encoding a TIC6281 pesticidal protein.
atgtcaaatcaagatttacagatggaaagctggttaacattaaatgatgtttcccttcatcaaaatattcaaacaccactttctttcgaccttacttcctctttacaagatgctgcacctgtccaagatactataagtggaggtttaattattggtaacacacaaaacgaagctatcgatgccagtaataatgtaaaaaatgcactgcaaacatacggtcgttttagtaatgaggtcaaagaatctgctcaagtaagtccgattgttggattaacaactatacttgatattgcaagaatagtttccaattacaacccggctttgcccactgatcaagaaaatgatgaaactaaaaaagcaagagttattgcatacaaccaatatattacgaaggtgttgcaaaatcctttaatgcacttaaaaagcaactatgaaaaaaaatacacaaaacgaacttctaactggaagacagctattgatgaaatcagtaatttatatgatggcatcacagaaaaagataaagagaaaattaaaaatagtttacaagctttagcagaagctgcttcttcaagatcaaatcaagccaatacagaaaatatatttgctcaaaatgttattgtgtgcaataatgaagaaattgaattttgtatttattcaagttcagttacaatgctttatagtggtggtaaaaataccgtaagacaggttgatttcactctaaacgaaacccacattagatttacaaaagagttatggagtagatactctgataaagttttagataaacacttagcgttgatagatgattggctacttggaattagtactcctaatagtgataaaactactctcgcttgctttgtttaa

SEQ ID NO: 25 - protein, 288 aa, Lysinibacillus sphaericus
  MISC_FEATURE (1)..(288): Amino acid sequence of the TIC6281 protein.
MSNQDLQMESWLTLNDVSLHQNIQTPLSFDLTSSLQDAAPVQDTISGGLIIGNTQNEAIDASNNVKNALQTYGRFSNEVKESAQVSPIVGLTTILDIARIVSNYNPALPTDQENDETKKARVIAYNQYITKVLQNPLMHLKSNYEKKYTKRTSNWKTAIDEISNLYDGITEKDKEKIKNSLQALAEAASSRSNQANTENIFAQNVIVCNNEEIEFCIYSSSVTMLYSGGKNTVRQVDFTLNETHIRFTKELWSRYSDKVLDKHLALIDDWLLGISTPNSDKTTLACFV

SEQ ID NO: 26 - DNA, 867 bp, Lysinibacillus sphaericus
  misc_feature (1)..(867): Nucleic acid sequence obtained from the Lysinibacillus sphaericus species AG0069H08 encoding a TIC6282 pesticidal protein.
atgtcaaatcaagatttacagatggaaagctggttaacagtaaatgatgtttcccttcatcaaaatattcaaacaccactttctttcgaccttacatcctctttacaagatgctgcacctgtccaagatactataagtggaggtttaattattggtaacacacaaaacgaagctatcgatgccaataataatgtaaaaaatgcactgcaaacatacggtcgttttagtaatgaggtcaaagaatctgctcaagtaagtccgattgttggattaacaactatacttgatattgcaagaatagtttccaattacaacccggctttgcccactgatcaagaaaatgatgaaactaaaaaagcaagagttattgcatacaaccaatatattacgaaggtgttgcaaaatcctttaatgcacttaaaaagcaactatgaaaaaaaatacacaaaacgaacttctaactggaagacagctattgaggaaatcagtaatttatatgatggcatcacagaaaaagataaagagaaaattaaaaatagtttacaagctttagcagaagctgcctcttcaagatcaaatcaagccaatacagaaaatatatttgctcaaaatgttattgtgtgcaatgatgaagaaattgaattttgtatttattcaagttcagttacaatgctttatagtggtggtaaaaataccgtaagacaggttgatttcactctaaacgaaacccacattagatttacaaaagagttatggagtagatactctgataaagttttagataaacacttagcgttgatagatgattggctacttggaattagtactcctaatagtgataaaactactctcgcttgctttgtttaa

SEQ ID NO: 27 - protein, 288 aa, Lysinibacillus sphaericus
  MISC_FEATURE (1)..(288): Amino acid sequence of the TIC6282 protein.
MSNQDLQMESWLTVNDVSLHQNIQTPLSFDLTSSLQDAAPVQDTISGGLIIGNTQNEAIDANNNVKNALQTYGRFSNEVKESAQVSPIVGLTTILDIARIVSNYNPALPTDQENDETKKARVIAYNQYITKVLQNPLMHLKSNYEKKYTKRTSNWKTAIEEISNLYDGITEKDKEKIKNSLQALAEAASSRSNQANTENIFAQNVIVCNDEEIEFCIYSSSVTMLYSGGKNTVRQVDFTLNETHIRFTKELWSRYSDKVLDKHLALIDDWLLGISTPNSDKTTLACFV

SEQ ID NO: 28 - DNA, 867 bp, Lysinibacillus sphaericus
  misc_feature (1)..(867): Nucleic acid sequence obtained from the Lysinibacillus sphaericus species AG0025E04 encoding a TIC6283 pesticidal protein.
atgtcaaatcaagatttacagatggaaagctggttaacagtaaatgatgtttcccttcatcaaaatattcaaacaccactttctttcgaccttacatcctctttacaagatgttgcacctgtccaagatactataagtggaggtttaattattggtaacacacaaaacgaagctatcgatgccaataataatgtaaaaaatgcactgcaaacatacggtcgttttagtaatgaggtcaaagaatctgctcaagtaagtccgattgttggattaacaactatacttgatattgcaagaatagtttccaattacaacccggctttgcccactgatcaagaaaatgatgaaactaaaaaagcaagagttattgcatacaaccaatatattacgaaggtgttgcaaaatcctttaatgcacttaaaaagcaactatgaaaaaaattacacaaaacgaacttctaactggaagacagctattgaggaaatcagtaatttatatgatggcatcacagaaaaagataaagagaaaattaaaaatagtttacaagctttagcagaagctgcctcttcaagatcaaatcaagccaatacagaaaatatatttgctcaaaatgttattgtgtgcaatgatgaagaaattgaattttgtatttattcaagttcagttacaatgctttatagtggtggtaaaaataccgtaagacaggttgatttcactctaaacgaaacccacattagatttacaaaagagttatggagtagatactctgataaagttttagataaacacttagcgttgatagatgattggctacttggaattagtactcctaatagtgataaaactactctcgcttgctttgtttaa

SEQ ID NO: 29 - protein, 288 aa, Lysinibacillus sphaericus
  MISC_FEATURE (1)..(288): Amino acid sequence of the TIC6283 protein.
MSNQDLQMESWLTVNDVSLHQNIQTPLSFDLTSSLQDVAPVQDTISGGLIIGNTQNEAIDANNNVKNALQTYGRFSNEVKESAQVSPIVGLTTILDIARIVSNYNPALPTDQENDETKKARVIAYNQYITKVLQNPLMHLKSNYEKNYTKRTSNWKTAIEEISNLYDGITEKDKEKIKNSLQALAEAASSRSNQANTENIFAQNVIVCNDEEIEFCIYSSSVTMLYSGGKNTVRQVDFTLNETHIRFTKELWSRYSDKVLDKHLALIDDWLLGISTPNSDKTTLACFV

SEQ ID NO: 30 - DNA, 825 bp, Lysinibacillus sphaericus
  misc_feature (1)..(825): Nucleic acid sequence obtained from the Lysinibacillus sphaericus species EGBS0420 encoding a TIC7016 pesticidal protein.
atgacaaatcttgacttaaaaatggaaagttggttagcactaaatgatatttctctacatcaaaatttagagcctgttgctattaaactcgcaacatcagatcaaacagttgtcagtcaaggaatctttgtagggaatcagttgtcggaggctagaattgctgacaatcaggttcagcaggcacttcaaagctttggacgctatagtactgctgtaaaagaagctgctaaagtagctccaacaactggtttaacaactatccttgacattgctagaatcgtttctaatttcaatccggcattaccaaacgataaaaataatgtacctgcctatgaaaaatatgtttcaaaaatattacaaaacccacttatccatttattaaatagcagtgtaaaatccttcaaacgtacgacttctgattggaatgaagcaattgaccaaattgccaatttatataatggcatttcggcagctgacaaaggaaaaattgtagaaagcttaaaagcattagcaaaatccgcctcctcttctagctctgaaaaacaaacggaaaaactatttactcaaagtacgattaactgtgaggaaaatatagatatttatatttactctagctctgtcacaatggaggagcacaacggtaagcacaatgtaaagcaggttgaatttgaaatacaagaaacacaattaagatttacaaaagaattgtggagtttatactctgatgctgtgttagctaaacatctagctctaatggatgattggctaaatggcattgatacaaaagcagacaatcgtttatccactcttacatgcttagtttaa

SEQ ID NO: 31 - protein, 274 aa, Lysinibacillus sphaericus
  MISC_FEATURE (1)..(274): Amino acid sequence of the TIC7016 protein.
MTNLDLKMESWLALNDISLHQNLEPVAIKLATSDQTVVSQGIFVGNQLSEARIADNQVQQALQSFGRYSTAVKEAAKVAPTTGLTTILDIARIVSNFNPALPNDKNNVPAYEKYVSKILQNPLIHLLNSSVKSFKRTTSDWNEAIDQIANLYNGISAADKGKIVESLKALAKSASSSSSEKQTEKLFTQSTINCEENIDIYIYSSSVTMEEHNGKHNVKQVEFEIQETQLRFTKELWSLYSDAVLAKHLALMDDWLNGIDTKADNRLSTLTCLV

SEQ ID NO: 32 - DNA, 825 bp, Lysinibacillus sphaericus
  misc_feature (1)..(825): Nucleic acid sequence obtained from the Lysinibacillus sphaericus species EGBS1094 encoding a TIC7017 pesticidal protein.
atgacaaatcttgacttaaaaatggaaagttggttagcactaaatgatatttctctacatcaaaatttagagcctgttgctattaaactcgcaacatcagatcaaacagttgtcagtcaaggaatctttgttgggaatcagctgtcggaggctagaattgctgacaaccaagttcagcaagcacttcaaagctttggacgctatagtgctgctgtaaaagaagctgctaaaatagctccaacaactggattaacaactatccttgacattgctagaattgtttctaatttcaatcctgcattaccaaacgataaaaataatgtacctgcctatgaaaaatatgtttcaaaaatattacaaaacccacttatccatttattaaatagcagtgtaaaatcctttaaacgtacgacttccgattggaatgaagcaattgaccaaattgccaatttatataatggcatttcggcagctgacaaaggaaaaattgtagaaagcttaaaagcattagcaaaatccgcctcttcttctagctctgaaaaacaaacggaaaaactatttactcaaagtacgattaactgtgaggaaaatattgatatttatatttactctagctctgtcacaatggaggagcacagcggtaagcataatgtaaagcaggttgaatttgaaatacaagaaacacaattaagatttacaaaagaattgtggagtttatactcagatgctgtgttagctaaacatctagcattaatggatgattggctgaatggcattgatacaaaagcagacaaccgtttatccactcttacatgcttagtttaa

SEQ ID NO: 33 - protein, 274 aa, Lysinibacillus sphaericus
  MISC_FEATURE (1)..(274): Amino acid sequence of the TIC7017 protein.
MTNLDLKMESWLALNDISLHQNLEPVAIKLATSDQTVVSQGIFVGNQLSEARIADNQVQQALQSFGRYSAAVKEAAKIAPTTGLTTILDIARIVSNFNPALPNDKNNVPAYEKYVSKILQNPLIHLLNSSVKSFKRTTSDWNEAIDQIANLYNGISAADKGKIVESLKALAKSASSSSSEKQTEKLFTQSTINCEENIDIYIYSSSVTMEEHSGKHNVKQVEFEIQETQLRFTKELWSLYSDAVLAKHLALMDDWLNGIDTKADNRLSTLTCLV

SEQ ID NO: 34 - DNA, 825 bp, Lysinibacillus sphaericus
  misc_feature (1)..(825): Nucleic acid sequence obtained from the Lysinibacillus sphaericus species AG0025E04 encoding a TIC7107 pesticidal protein.
atgacaaatcttgacttaaaaatggaaagctggttagcactaaatgatatttctctgcatcaaaatttagagcctgttgctattaaacttgctccatcagatcaaacagttgtcagtcaaggaatctttgttgggagtcagctgtcggaggctagaatcgctgacaatcaagttcagcaagcacttcaaaactttggacgctatagttctgcggtaaaagaagctgctaaagtagctccaacaactggattaacaactattcttgacattgctagaattgtctctaattttaatccagcattaccaaacgataaaaataatgttcctgcttatgaaaaatatgtgtcaaaaattttacaaaacccacttatccatttattaaatagcagtctaaaatcctttaaacgtaggacttccgattggaatgaagtaattgaccaaatcgccaatttatataatggcatttcggcagttgataaaggaaaaatcgtagaaagcttaaaagcattagcaaattccgcctcttcttctagctcagaaaaacaaactgaaaaactatttactcaaagcacgattaactgtgaggaaaatattgatatttatatttactctagctctgttacaatggaggagcacaatgggaagcataatgtaaaacaagttgaatttgaaatacaagaaacacaattaagatttacaaaagaattgtggagtttatactcagatgctgtgttagcaaaacatctagctttaatggatgattggctcaatggcattgatacaaaagctgacaatcgtttatccactcttacatgcttagtttag

SEQ ID NO: 35 - DNA, 825 bp, Lysinibacillus sphaericus
  misc_feature (1)..(825): Nucleic acid sequence obtained from the Lysinibacillus sphaericus species AG0067H01 encoding a TIC7108 pesticidal protein.
atgacaaatcttgacttaaaaatggaaagctggttagcactaaatgatatttctctgcatcaaaatttagagcctgttgctattaaacttgcaccatcagatcaaacagttgtcagtcaaggaatctttgttgggagtcagctgtcggaggctagaatcgctgacaatcaagttcagcaagcacttcaaaactttggacgctatagttctgcagtaaaagaagctgctaaagtagctccaacaactggattaacaactattcttgatattgctagaattgtttctaattttaatccagcattaccaaacgataaaaataatgttcctgcttatgaaaaatatgtgtcaaaaattttacaaaacccacttatccatttattaaatagcagtctaaaatcctttaaacgtaggacttccgattggaatgaagtaattgaccaaatcgccaatttatataatggcatttcggcagttgataaaggaaaaatcgtagaaagcttaaaagcattagcaaattccgcctcttcttctagctcagaaaaacaaattgaaaaactatttactcaaagcacgattaactgtgaggaaaatattgatatttatatttactctagctctgttacaatggaggagcacaatgggaagcataatgtaaagcaagttgaatttgaaatacaagaaacacaattaagatttacaaaagaattgtggagtttatactcagatgctgtgttagcaaaacatctagctttaatggatgattggctcaatggcattgatacaaaagctgacaatcgtttatccactcttacatgcttagtttag

SEQ ID NO: 36 - protein, 274 aa, Lysinibacillus sphaericus
  MISC_FEATURE (1)..(274): Amino acid sequence of the TIC7108 protein.
MTNLDLKMESWLALNDISLHQNLEPVAIKLAPSDQTVVSQGIFVGSQLSEARIADNQVQQALQNFGRYSSAVKEAAKVAPTTGLTTILDIARIVSNFNPALPNDKNNVPAYEKYVSKILQNPLIHLLNSSLKSFKRRTSDWNEVIDQIANLYNGISAVDKGKIVESLKALANSASSSSSEKQIEKLFTQSTINCEENIDIYIYSSSVTMEEHNGKHNVKQVEFEIQETQLRFTKELWSLYSDAVLAKHLALMDDWLNGIDTKADNRLSTLTCLV

SEQ ID NO: 37 - DNA, 825 bp, Lysinibacillus sphaericus
  misc_feature (1)..(825): Nucleic acid sequence obtained from the Lysinibacillus sphaericus species AG0067H03 encoding a TIC7109 pesticidal protein.
atgacaaatcttgacttaaaaatggaaagctggttagcactaaatgatatttctctgcatcaaaatttagagcctgttgctattaaacttgcaccatcagatcaaacagttgtcagtcaaggaatctttgttgggagtcagctgtcggaggctagaatcgctgacaatcaagttcagcaagcacttcaaaactttggacgctatagttctgcagtaaaagaagctgctaaagtagctccaacaactggattaacaactattcttgatattgctagaattgtttctaattttaatccagcattaccaaacgataaaaataatgttcctgcttatgaaaaatatgtgtcaaaaattttacaaaacccacttatccatttattaaatagcagtctaaaatcctttaaacgtaggacttccgattggaatgaagtaattgaccaaatcgccaatttatataatggcatttcggcagttgataaaggaaaaatcgtagaaagcttaaaagcattagcaaattccgcctcttcttctagctcagaaaaacaaactgaaaaactatttactcaaagcacgattaactgtgaggaaaatattgatatttatatttactctagctctgttacaatggaggagcacaatgggaagcataatgtaaagcaagttgaatttgaaatacaagaaacacaattaagatttacaaaagaattgtggagtttatactcagatgctgtgttagcaaaacatctagctttaatggatgattggctcaatggcattgatacaaaagctgacaatcgtttatccactcttacatgcttagtttag

SEQ ID NO: 38 - DNA, 825 bp, Lysinibacillus sphaericus
  misc_feature (1)..(825): Nucleic acid sequence obtained from the Lysinibacillus sphaericus species AG0067H07 encoding a TIC7110 pesticidal protein.
atgacaaatcttgacttaaaaatggaaagctggttagcactaaatgatatttctctgcatcaaaatttagagcctgttgctattaaacttgcaccatcagatcaaacagttgtcagtcaaggaatctttgttgggagtcagctgtcggaggctagaatcgctgacaatcaagttcagcaagcacttcaaaactttggacgctatagttctgcagtaaaagaagctgctaaagtagctccaacaactggattaacaactattcttgatattgctagaattgtttctaattttaatccagcattaccaaacgataaaaataatgttcctgcttatgaaaaatatgtgtcaaaaattttacaaaacccacttatccatttattaaatagcagtctaaaatcctttaaacgtaggacttccgattggaatgaagtaattgaccaaatcgccaatttatataatggcatttcggcagttgataaaggaaaaatcgtagaaagcttaaaagcattagcaaattccgcctcttcttctagctcagaaaaacaaactgaaaaactatttactcaaagcacgattaactgtgaggaaaatattgatatttatatttactctagctctgttacaatggaggagcacaatgggaagcataatgtaaagcaagttgaatttgaaatacaagaaactcaattaagatttacaaaagaattgtggagtttatactcagatgctgtgttagcaaaacatctagctttaatggatgattggctcaatggcattgatacaaaagctgacaatcgtttatccactcttacatgcttagtttag

SEQ ID NO: 39 - protein, 274 aa, Lysinibacillus sphaericus
  MISC_FEATURE (1)..(274): Amino acid sequence of the TIC7110 protein.
MTNLDLKMESWLALNDISLHQNLEPVAIKLAPSDQTVVSQGIFVGSQLSEARIADNQVQQALQNFGRYSSAVKEAAKVAPTTGLTTILDIARIVSNFNPALPNDKNNVPAYEKYVSKILQNPLIHLLNSSLKSFKRRTSDWNEVIDQIANLYNGISAVDKGKIVESLKALANSASSSSSEKQTEKLFTQSTINCEENIDIYIYSSSVTMEEHNGKHNVKQVEFEIQETQLRFTKELWSLYSDAVLAKHLALMDDWLNGIDTKADNRLSTLTCLV

SEQ ID NO: 40 - DNA, 825 bp, Lysinibacillus sphaericus
  misc_feature (1)..(825): Nucleic acid sequence obtained from the Lysinibacillus sphaericus species AG0069H08 encoding a TIC7111 pesticidal protein.
atgacaaatcttgacttaaaaatggaaagctggttagcactaaatgatatttctctgcatcaaaatttagagcctgttgctattaaacttgcaccatcagatcaaacagttgtcagtcaaggaatctttgttgggagtcagctgtcggaggctagaatcgctgacaatcaagttcagcaagcacttcaaaactttggacgctatagttctgcagtaaaagaagctgctaaagtagctccaacaactggattaacaactattcttgacattgctagaattgtctctaattttaatccagcattaccaaacgataaaaataatgttcctgcttatgaaaaatatgtgtcaaaaattttacaaaacccacttatccatttattaaatagcagtctaaaatcctttaaacgtaggacttccgattggaatgaagtaattgaccaaatcgccaatttatataatggcatttcggcagttgataaaggaaaaatcgtagaaagcttaaaagcattagcaaattccgcctcttcttctagctcagaaaaacaaactgaaaaactatttactcaaagcacgattaactgtgaggaaaatattgatatttatatttactctagctctgttacaatggaggagcacaatgggaagcataatgtaaagcaagttgaatttgaaatacaagaaacacaattaagatttacaaaagaattgtggagtttatactcagatgctgtgttagcaaaacatctagctttaatggatgattggctcaatggcattgatacaaaagctgacaatcgtttatccactcttacatgcttagtttag

SEQ ID NO: 41 - DNA, 828 bp, Lysinibacillus sphaericus
  misc_feature (1)..(828): Nucleic acid sequence obtained from the Lysinibacillus sphaericus species AG0122F12 encoding a TIC7589 pesticidal protein.
atgacaaatcttgatttaaaaatggaaagttggttggctgtaaatgatgtttctcaccaccagaatcttcaacaaccatattctgagatttcatcaacatctgaagaagtacttgtaagtcaaggattatttgtaggtgataaattggaaaacgcaataagtgcagataccaatgtccaacaagcacttcaaacatacggtcgttatagcgacgcagtaaaagaagcaactaaacttgcaccaacaaccggcttaacaacgttacttgatatttcacgaattgtttctggctttaatccagatttacctaatgatcctaaaaatgtccaagcatacaatcaatacattacaacaatattgaaaaatcctctttttcatttactaaaatctgaaagagtaaagtttacgagagctacatcagactggaatgaagcaattgataaaattgcggatctttatgatggtatacctacatctgataaaagtaagattgtaaaaagcttaaagacattagcagaagccgcctcttcttataccgaaaccaaccaaacagattatttatttacccaaagtacagtaaattgcagtgacaatattgatgtttatatttactcaagtacagtgacattgaaagaaaaaagtgggaaacatcacgtaaaagaatctacccttgatataggctgcgtacaattaagatttacaaaagagttatggagtgtatactctgatgaagtcttaaaaagacatttagcgttgatgactgattggttaaatgccatgaattcgaaaccaggaactaaacaatcgaaactcacttgcttagtttaa

SEQ ID NO: 42 - protein, 275 aa, Lysinibacillus sphaericus
  MISC_FEATURE (1)..(275): Amino acid sequence of the TIC7589 protein.
MTNLDLKMESWLAVNDVSHHQNLQQPYSEISSTSEEVLVSQGLFVGDKLENAISADTNVQQALQTYGRYSDAVKEATKLAPTTGLTTLLDISRIVSGFNPDLPNDPKNVQAYNQYITTILKNPLFHLLKSERVKFTRATSDWNEAIDKIADLYDGIPTSDKSKIVKSLKTLAEAASSYTETNQTDYLFTQSTVNCSDNIDVYIYSSTVTLKEKSGKHHVKESTLDIGCVQLRFTKELWSVYSDEVLKRHLALMTDWLNAMNSKPGTKQSKLTCLV

SEQ ID NO: 43 - DNA, 867 bp, Artificial
  Synthetic coding sequence encoding a TIC6280 pesticidal protein designed for expression in a plant cell.
atgagcaatcaggatctccagatggagtcctggctgaccctgaacgatgtgtccctacaccagaacatccagacgccgctgtcgttcgacctgacctcctcgctccaggacgccgcgccggtccaggacaccatctcaggcggcctcatcatcggcaacacgcagaacgaggccatcgacgccaacaacaacgtaaagaacgccttgcagacctacgggcgtttctccaacgaggtgaaggagtcggcccaagtcagccctatcgtgggcctcacgactatcttggacatcgccagaattgtctccaactacaacccggccctgcccacggaccaggagaacgacgagacgaagaaggcgcgggtcattgcgtacaaccagtacatcacgaaagtcttgcagaatcccttaatgcacctcaagtccaactacgagaagaagtacacgaagcggaccagtaactggaagacggccatcgacgaaatctccaacctctacgacggtatcacggagaaggacaaggagaagatcaagaactcgctccaggcgctcgccgaggcggccagctcccggtccaaccaggcgaacacggagaacatcttcgcgcagaacgtgatcgtgtgcaacgacgaggagatcgagttctgcatctactccagcagtgtgacgatgctctattctggcggcaagaacaccgtgcggcaagtggacttcacattgaacgagacgcacatccgcttcacgaaggagctgtggtctcgctactcggacaaggtgctcgacaagcacttggcgctgatcgacgactggctgctgggcatctccacgcccaactcagacaagaccacactggcgtgcttcgtgtga

SEQ ID NO: 44 - DNA, 867 bp, Artificial
  Synthetic coding sequence encoding a TIC6282 pesticidal protein designed for expression in a plant cell.
atgagcaaccaggatctccagatggagtcctggcttactgtgaatgacgtgagcctgcaccagaacatccagacgccgctcagcttcgacctcacctccagtctccaggacgccgcgccggtccaggacaccatctctggcggcctcatcatcggcaacacgcagaacgaggccatcgacgcgaacaataacgtcaagaacgccctccaaacctacggccgcttctccaacgaggtcaaagagtccgcccaagtgtcgcccatcgtcggtttaaccaccatcctggacatcgcccgcatcgtctcgaactacaacccggcgctgccgaccgaccaggagaacgacgagacgaagaaggccagggtgatcgcctacaaccagtacatcaccaaggtgctccagaacccgctcatgcacctcaagtcgaactacgagaagaagtacaccaagcgcacaagcaactggaagaccgccatcgaggagatcagcaacttgtacgacggcatcacggagaaggacaaggagaagatcaagaacagtttacaggccctagccgaagccgcctcttcccgaagcaaccaggccaacaccgagaacatcttcgcgcagaacgtgatcgtgtgcaacgacgaggagatcgagttctgcatctactcctccagcgtgaccatgctctacagcggcggcaagaacaccgtacgacaagtggatttcacgctgaacgagactcacatccggttcacgaaggaactctggtcgcgctacagcgacaaggtgctggacaagcacttggcgctcatcgacgactggctgctgggcatcagcacgcccaatagtgacaagacgaccctcgcgtgcttcgtgtga

SEQ ID NO: 45 - DNA, 867 bp, Artificial
  Synthetic coding sequence encoding a TIC6283 pesticidal protein designed for expression in a plant cell.
atgtcgaaccaggatctccagatggagtcgtggcttacggtgaatgatgtgtcgctgcaccagaacatacaaacgccgctcagcttcgacctcacgtcgtccctccaggacgtggctcccgtgcaagacacgattagcggcgggctcatcatcggcaacacgcagaacgaggcgatagacgccaacaacaacgtcaagaacgccctccagacctacggccggttcagcaacgaggtgaaggagtcggcccaagtctcgcccatcgtcggcctcacgactatcctggacatcgcccgtatcgtctcgaactacaacccggcgctcccgaccgaccaggagaacgacgagaccaagaaggcccgcgtgatcgcgtacaaccagtacatcaccaaggtgctccagaacccgctgatgcacctcaagtcgaactacgagaagaactacactaagcggacttccaactggaagaccgccatcgaggaaatctcgaacctgtacgacggcatcaccgagaaggacaaggagaagataaagaacagcctccaggccctcgcggaggcggcctcgtcccgctccaaccaggctaataccgagaacatcttcgcccagaacgtcattgtgtgtaacgacgaggagattgagttctgcatctacagcagcagcgtgaccatgctgtactcaggcgggaagaatacggtgcgccaagtggacttcacgctgaacgagacccacatccgcttcaccaaggagctgtggtcccgatactccgacaaggtgctcgacaagcacctcgcgctcatcgacgactggctgctgggcatctccacgccgaacagcgacaagaccacgctcgcctgcttcgtgtag

SEQ ID NO: 46 - DNA, 828 bp, Artificial
  Synthetic coding sequence encoding a TIC7016PL pesticidal protein designed for expression in a plant cell, wherein an additional codon encoding an alanine residue is inserted immediately following the initiating methionine codon.
atggctacaaacctcgacctcaagatggagagctggctggcgctcaacgacatcagtctccaccagaacctcgagccggtcgctatcaaactcgctacctccgaccaaaccgtggtgtcccagggcatcttcgtcggcaaccagctcagcgaggcccggatcgccgacaaccaggtccaacaggccctgcagagtttcgggcggtacagcacggcagtcaaagaggccgcgaaggtggctccgaccaccgggctgactaccatcctggacatcgcgcggatcgtctcgaacttcaatccggctctgccgaacgacaagaacaacgttcccgcctacgagaagtacgtttcgaagatcctgcagaacccactgatacacctgctcaattcgtccgtgaagtctttcaagcgcactacgtcggactggaacgaagcgatcgaccagatcgccaacctgtacaacggcatcagtgccgcggacaagggcaagatcgtcgagagcctcaaggccctcgcaaagtcggcctccagctctagcagcgagaaacagaccgagaagctcttcacccagagcaccatcaactgcgaggagaacatcgacatctacatctactcctcgtccgtgacaatggaggagcacaacggcaagcacaatgtgaagcaagtggagttcgagatccaggagacgcagctccgcttcaccaaggagctctggagcctctactctgacgcagtgttggcaaagcacctcgctttgatggacgactggcttaacgggatcgacactaaagcggacaacagactgagcaccctcacctgcctggtctga

SEQ ID NO: 47 - protein, 275 aa, Artificial
  Amino acid sequence of TIC7016PL, wherein an additional alanine residue is inserted immediately following the initiating methionine.
MATNLDLKMESWLALNDISLHQNLEPVAIKLATSDQTVVSQGIFVGNQLSEARIADNQVQQALQSFGRYSTAVKEAAKVAPTTGLTTILDIARIVSNFNPALPNDKNNVPAYEKYVSKILQNPLIHLLNSSVKSFKRTTSDWNEAIDQIANLYNGISAADKGKIVESLKALAKSASSSSSEKQTEKLFTQSTINCEENIDIYIYSSSVTMEEHNGKHNVKQVEFEIQETQLRFTKELWSLYSDAVLAKHLALMDDWLNGIDTKADNRLSTLTCLV

SEQ ID NO: 48 - DNA, 828 bp, Artificial
  Synthetic coding sequence encoding a TIC7017PL pesticidal protein designed for expression in a plant cell, wherein an additional codon encoding an alanine residue is inserted immediately following the initiating methionine codon.
atggctacgaacctggatctcaagatggagtcatggctggcgctcaacgacatcagcctgcaccagaatctcgagccggttgccatcaagctggccacctccgaccagacggtcgtgtcccagggcatctttgtgggcaaccagctgtccgaggcgcggatagcggacaaccaggtccagcaagcgctgcaatccttcggtcgatacagcgccgccgtgaaggaggcagccaagatcgcgccaacaaccggcctcaccacgatactggacattgcccgcattgtctccaatttcaacccggcccttccgaacgacaagaacaacgtgccggcatacgagaagtacgtctccaaaatcttacagaatcctctcatccacctcctgaatagcagcgtcaagagtttcaagcgcaccacgagtgactggaacgaggcgatcgaccagatcgcgaacctttacaatggaatcagcgccgccgacaagggcaagatcgtggagagtctcaaggcgctggcgaagtccgcctccagcagttccagcgagaagcagacggagaagctgttcacccagagcaccatcaactgcgaggagaacatcgacatctacatctacagcagctcggtcacgatggaggagcactcagggaagcacaacgtcaagcaagtggagttcgagatccaggagacccagctccgcttcacaaaggaactgtggagcctttactccgacgccgtcctggcaaagcacctcgcgctcatggacgactggctgaacggcatcgacaccaaggcggacaaccggctgagcaccctaacctgcctcgtctga

SEQ ID NO: 49 - protein, 275 aa, Artificial
  Amino acid sequence of TIC7017PL, wherein an additional alanine residue is inserted immediately following the initiating methionine.
MATNLDLKMESWLALNDISLHQNLEPVAIKLATSDQTVVSQGIFVGNQLSEARIADNQVQQALQSFGRYSAAVKEAAKIAPTTGLTTILDIARIVSNFNPALPNDKNNVPAYEKYVSKILQNPLIHLLNSSVKSFKRTTSDWNEAIDQIANLYNGISAADKGKIVESLKALAKSASSSSSEKQTEKLFTQSTINCEENIDIYIYSSSVTMEEHSGKHNVKQVEFEIQETQLRFTKELWSLYSDAVLAKHLALMDDWLNGIDTKADNRLSTLTCLV

SEQ ID NO: 50 - DNA, 828 bp, Artificial
  Synthetic coding sequence encoding a TIC7108PL pesticidal protein designed for expression in a plant cell, wherein an additional codon encoding an alanine residue is inserted immediately following the initiating methionine codon.
atggctaccaacctcgaccttaagatggagtcgtggttggcgctgaacgacatctccctccatcagaatctcgagccagtggccatcaagctggcgccctccgaccagactgtcgtgtcccagggcatcttcgtgggctcccaactgagcgaggcgcggatcgccgacaaccaggtgcagcaagcgctgcagaacttcggccgctacagctccgctgtgaaggaggccgccaaggtcgctcctaccaccggcctcaccactattctcgacattgccagaatcgtctccaacttcaacccggcgctcccgaacgacaagaacaacgtcccggcctacgagaagtacgtctcgaagattcttcagaacccgctcatccacctcctgaacagcagcctcaagtcattcaagcgccgcaccagcgactggaacgaggtcatcgaccagattgcgaacctctacaacggcatcagcgcagtggataagggcaagatcgtcgagtccctcaaggccctggcgaacagtgcctcttccagctcttccgagaagcagatcgagaagctctttacccaaagcacgattaactgcgaggagaacatcgacatctacatctactcatcatccgtgacgatggaggagcacaatggcaagcacaacgtgaagcaagtggagttcgagatccaggagacccagctccggttcaccaaggagctatggtccctctactcggacgcggtcctcgccaaacacctggcgctcatggacgactggctgaatggaatagacactaaggcggacaaccggctctccacgctcacgtgcctcgtctga

SEQ ID NO: 51 - protein, 275 aa, Artificial
  Amino acid sequence of TIC7108PL, wherein an additional alanine residue is inserted immediately following the initiating methionine.
MATNLDLKMESWLALNDISLHQNLEPVAIKLAPSDQTVVSQGIFVGSQLSEARIADNQVQQALQNFGRYSSAVKEAAKVAPTTGLTTILDIARIVSNFNPALPNDKNNVPAYEKYVSKILQNPLIHLLNSSLKSFKRRTSDWNEVIDQIANLYNGISAVDKGKIVESLKALANSASSSSSEKQIEKLFTQSTINCEENIDIYIYSSSVTMEEHNGKHNVKQVEFEIQETQLRFTKELWSLYSDAVLAKHLALMDDWLNGIDTKADNRLSTLTCLV

SEQ ID NO: 52 - DNA, 828 bp, Artificial
  Synthetic coding sequence encoding a TIC7110PL pesticidal protein designed for expression in a plant cell, wherein an additional codon encoding an alanine residue is inserted immediately following the initiating methionine codon.
atggctaccaacctcgacctcaagatggagtcctggctcgcgctgaatgacatctcgctgcaccagaatctggagcccgtcgccatcaagctcgcgcccagcgaccagacagttgtttcccagggcatcttcgtgggcagccagctcagcgaagcgcgtatcgccgacaaccaggtgcagcaagccctgcagaacttcgggcggtactccagcgcggtgaaggaggcggcgaaggtcgctccgactacagggctcacaaccattctcgacatcgcgcgcatcgtctcgaacttcaacccggctctcccgaacgacaagaacaacgtcccggcttacgagaagtacgtcagcaagatcctccagaacccgctgatccacttactcaattctagcctcaaatcctttaaacgacggacctccgattggaacgaggtgatcgaccagattgcgaacctttacaacggcatctctgccgttgacaagggcaagatcgtcgagtcactcaaagcgctggcgaatagcgccagctcctcatcttctgagaagcagactgagaagctctttacccagtccacgatcaactgcgaggagaacatcgacatctacatctactccagcagcgtcacgatggaggagcacaatggcaagcacaacgtgaagcaagtggagttcgagatccaggagacccagctccggttcactaaggagctttggtcgctctactcggacgccgtgctggcgaagcacctggcgctgatggacgactggctgaacgggatagacacgaaggccgacaaccgcctgagtaccttgacctgcttggtctga

SEQ ID NO: 53 - protein, 275 aa, Artificial
  Amino acid sequence of TIC7110PL, wherein an additional alanine residue is inserted immediately following the initiating methionine.
MATNLDLKMESWLALNDISLHQNLEPVAIKLAPSDQTVVSQGIFVGSQLSEARIADNQVQQALQNFGRYSSAVKEAAKVAPTTGLTTILDIARIVSNFNPALPNDKNNVPAYEKYVSKILQNPLIHLLNSSLKSFKRRTSDWNEVIDQIANLYNGISAVDKGKIVESLKALANSASSSSSEKQTEKLFTQSTINCEENIDIYIYSSSVTMEEHNGKHNVKQVEFEIQETQLRFTKELWSLYSDAVLAKHLALMDDWLNGIDTKADNRLSTLTCLV

SEQ ID NO: 54 - DNA, 1689 bp, Artificial
  Synthetic sequence encoding a TIC7110/TIC6280 fusion toxin protein, TIC7110-TIC6280F1, wherein the two toxin protein encoding sequences are contiguous and in frame.
atgacaaatcttgacttaaaaatggaaagctggttagcactaaatgatatttctctgcatcaaaatttagagcctgttgctattaaacttgcaccatcagatcaaacagttgtcagtcaaggaatctttgttgggagtcagctgtcggaggctagaatcgctgacaatcaagttcagcaagcacttcaaaactttggacgctatagttctgcagtaaaagaagctgctaaagtagctccaacaactggattaacaactattcttgatattgctagaattgtttctaattttaatccagcattaccaaacgataaaaataatgttcctgcttatgaaaaatatgtgtcaaaaattttacaaaacccacttatccatttattaaatagcagtctaaaatcctttaaacgtaggacttccgattggaatgaagtaattgaccaaatcgccaatttatataatggcatttcggcagttgataaaggaaaaatcgtagaaagcttaaaagcattagcaaattccgcctcttcttctagctcagaaaaacaaactgaaaaactatttactcaaagcacgattaactgtgaggaaaatattgatatttatatttactctagctctgttacaatggaggagcacaatgggaagcataatgtaaagcaagttgaatttgaaatacaagaaactcaattaagatttacaaaagaattgtggagtttatactcagatgctgtgttagcaaaacatctagctttaatggatgattggctcaatggcattgatacaaaagctgacaatcgtttatccactcttacatgcttagttatgtcaaatcaagatttacagatggaaagctggttaacattaaatgatgtttcccttcatcaaaatattcaaacaccactttctttcgaccttacttcctctttacaagatgctgcacctgtccaagatactataagtggaggtttaattattggtaacacacaaaacgaagctatcgatgccaataataatgtaaaaaatgcactgcaaacatacggtcgttttagtaatgaggtcaaagaatctgctcaagtaagtccgattgttggattaacaactatacttgatattgcaagaatagtttccaattacaacccggctttgcccactgatcaagaaaatgatgaaactaaaaaagcaagagttattgcatacaaccaatatattacgaaggtgttgcaaaatcctttaatgcacttaaaaagcaactatgaaaaaaaatacacaaaacgaacttctaactggaagacagctattgatgaaatcagtaatttatatgatggcatcacagaaaaagataaagagaaaattaaaaatagtttacaagctttagcagaagctgcttcttcaagatcaaatcaagccaatacagaaaatatatttgctcaaaatgttattgtgtgcaatgatgaagaaattgaattttgtatttattcaagttcagttacaatgctttatagtggtggtaaaaataccgtaagacaggttgatttcactctaaacgaaacccacattagatttacaaaagagttatggagtagatactctgataaagttttagataaacacttagcgttgatagatgattggctacttggaattagtactcctaatagtgataaaactactctcgcttgctttgtttaa

SEQ ID NO: 55 - protein, 562 aa, Artificial
  Amino acid sequence of a TIC7110/TIC6280 fusion toxin protein, TIC7110-TIC6280F1, wherein the two toxin protein amino acid sequences are contiguous.
MTNLDLKMESWLALNDISLHQNLEPVAIKLAPSDQTVVSQGIFVGSQLSEARIADNQVQQALQNFGRYSSAVKEAAKVAPTTGLTTILDIARIVSNFNPALPNDKNNVPAYEKYVSKILQNPLIHLLNSSLKSFKRRTSDWNEVIDQIANLYNGISAVDKGKIVESLKALANSASSSSSEKQTEKLFTQSTINCEENIDIYIYSSSVTMEEHNGKHNVKQVEFEIQETQLRFTKELWSLYSDAVLAKHLALMDDWLNGIDTKADNRLSTLTCLVMSNQDLQMESWLTLNDVSLHQNIQTPLSFDLTSSLQDAAPVQDTISGGLIIGNTQNEAIDANNNVKNALQTYGRFSNEVKESAQVSPIVGLTTILDIARIVSNYNPALPTDQENDETKKARVIAYNQYITKVLQNPLMHLKSNYEKKYTKRTSNWKTAIDEISNLYDGITEKDKEKIKNSLQALAEAASSRSNQANTENIFAQNVIVCNDEEIEFCIYSSSVTMLYSGGKNTVRQVDFTLNETHIRFTKELWSRYSDKVLDKHLALIDDWLLGISTPNSDKTTLACFV

SEQ ID NO: 56 - DNA, 1707 bp, Artificial
  Synthetic sequence encoding a TIC7110/TIC6280 fusion toxin protein, TIC7110-TIC6280F2, wherein a cleavable linker sequence (Linker 1) is operably linked and in frame between the two toxin protein encoding sequences.
atgacaaatcttgacttaaaaatggaaagctggttagcactaaatgatatttctctgcatcaaaatttagagcctgttgctattaaacttgcaccatcagatcaaacagttgtcagtcaaggaatctttgttgggagtcagctgtcggaggctagaatcgctgacaatcaagttcagcaagcacttcaaaactttggacgctatagttctgcagtaaaagaagctgctaaagtagctccaacaactggattaacaactattcttgatattgctagaattgtttctaattttaatccagcattaccaaacgataaaaataatgttcctgcttatgaaaaatatgtgtcaaaaattttacaaaacccacttatccatttattaaatagcagtctaaaatcctttaaacgtaggacttccgattggaatgaagtaattgaccaaatcgccaatttatataatggcatttcggcagttgataaaggaaaaatcgtagaaagcttaaaagcattagcaaattccgcctcttcttctagctcagaaaaacaaactgaaaaactatttactcaaagcacgattaactgtgaggaaaatattgatatttatatttactctagctctgttacaatggaggagcacaatgggaagcataatgtaaagcaagttgaatttgaaatacaagaaactcaattaagatttacaaaagaattgtggagtttatactcagatgctgtgttagcaaaacatctagctttaatggatgattggctcaatggcattgatacaaaagctgacaatcgtttatccactcttacatgcttagttggtagtggcggtgcttcaatgtcaaatcaagatttacagatggaaagctggttaacattaaatgatgtttcccttcatcaaaatattcaaacaccactttctttcgaccttacttcctctttacaagatgctgcacctgtccaagatactataagtggaggtttaattattggtaacacacaaaacgaagctatcgatgccaataataatgtaaaaaatgcactgcaaacatacggtcgttttagtaatgaggtcaaagaatctgctcaagtaagtccgattgttggattaacaactatacttgatattgcaagaatagtttccaattacaacccggctttgcccactgatcaagaaaatgatgaaactaaaaaagcaagagttattgcatacaaccaatatattacgaaggtgttgcaaaatcctttaatgcacttaaaaagcaactatgaaaaaaaatacacaaaacgaacttctaactggaagacagctattgatgaaatcagtaatttatatgatggcatcacagaaaaagataaagagaaaattaaaaatagtttacaagctttagcagaagctgcttcttcaagatcaaatcaagccaatacagaaaatatatttgctcaaaatgttattgtgtgcaatgatgaagaaattgaattttgtatttattcaagttcagttacaatgctttatagtggtggtaaaaataccgtaagacaggttgatttcactctaaacgaaacccacattagatttacaaaagagttatggagtagatactctgataaagttttagataaacacttagcgttgatagatgattggctacttggaattagtactcctaatagtgataaaactactctcgcttgctttgtttaa

SEQ ID NO: 57 - protein, 568 aa, Artificial
  Amino acid sequence of a TIC7110/TIC6280 fusion toxin protein, TIC7110-TIC6280F2,  wherein a cleavable linker peptide sequence (Linker 1) is inserted between the two toxin protein amino acid sequences.
MTNLDLKMESWLALNDISLHQNLEPVAIKLAPSDQTVVSQGIFVGSQLSEARIADNQVQQALQNFGRYSSAVKEAAKVAPTTGLTTILDIARIVSNFNPALPNDKNNVPAYEKYVSKILQNPLIHLLNSSLKSFKRRTSDWNEVIDQIANLYNGISAVDKGKIVESLKALANSASSSSSEKQTEKLFTQSTINCEENIDIYIYSSSVTMEEHNGKHNVKQVEFEIQETQLRFTKELWSLYSDAVLAKHLALMDDWLNGIDTKADNRLSTLTCLVGSGGASMSNQDLQMESWLTLNDVSLHQNIQTPLSFDLTSSLQDAAPVQDTISGGLIIGNTQNEAIDANNNVKNALQTYGRFSNEVKESAQVSPIVGLTTILDIARIVSNYNPALPTDQENDETKKARVIAYNQYITKVLQNPLMHLKSNYEKKYTKRTSNWKTAIDEISNLYDGITEKDKEKIKNSLQALAEAASSRSNQANTENIFAQNVIVCNDEEIEFCIYSSSVTMLYSGGKNTVRQVDFTLNETHIRFTKELWSRYSDKVLDKHLALIDDWLLGISTPNSDKTTLACFV

SEQ ID NO: 58 - DNA, 1728 bp, Artificial
  Synthetic sequence encoding a TIC7110/TIC6280 fusion toxin protein, TIC7110-TIC6280F3, wherein a flexible linker sequence (Linker 2) is operably linked and in frame between the two toxin protein encoding sequences.
atgacaaatcttgacttaaaaatggaaagctggttagcactaaatgatatttctctgcatcaaaatttagagcctgttgctattaaacttgcaccatcagatcaaacagttgtcagtcaaggaatctttgttgggagtcagctgtcggaggctagaatcgctgacaatcaagttcagcaagcacttcaaaactttggacgctatagttctgcagtaaaagaagctgctaaagtagctccaacaactggattaacaactattcttgatattgctagaattgtttctaattttaatccagcattaccaaacgataaaaataatgttcctgcttatgaaaaatatgtgtcaaaaattttacaaaacccacttatccatttattaaatagcagtctaaaatcctttaaacgtaggacttccgattggaatgaagtaattgaccaaatcgccaatttatataatggcatttcggcagttgataaaggaaaaatcgtagaaagcttaaaagcattagcaaattccgcctcttcttctagctcagaaaaacaaactgaaaaactatttactcaaagcacgattaactgtgaggaaaatattgatatttatatttactctagctctgttacaatggaggagcacaatgggaagcataatgtaaagcaagttgaatttgaaatacaagaaactcaattaagatttacaaaagaattgtggagtttatactcagatgctgtgttagcaaaacatctagctttaatggatgattggctcaatggcattgatacaaaagctgacaatcgtttatccactcttacatgcttagttggaagcggaacacatcaatctggtaagacatcgggatctatgtcaaatcaagatttacagatggaaagctggttaacattaaatgatgtttcccttcatcaaaatattcaaacaccactttctttcgaccttacttcctctttacaagatgctgcacctgtccaagatactataagtggaggtttaattattggtaacacacaaaacgaagctatcgatgccaataataatgtaaaaaatgcactgcaaacatacggtcgttttagtaatgaggtcaaagaatctgctcaagtaagtccgattgttggattaacaactatacttgatattgcaagaatagtttccaattacaacccggctttgcccactgatcaagaaaatgatgaaactaaaaaagcaagagttattgcatacaaccaatatattacgaaggtgttgcaaaatcctttaatgcacttaaaaagcaactatgaaaaaaaatacacaaaacgaacttctaactggaagacagctattgatgaaatcagtaatttatatgatggcatcacagaaaaagataaagagaaaattaaaaatagtttacaagctttagcagaagctgcttcttcaagatcaaatcaagccaatacagaaaatatatttgctcaaaatgttattgtgtgcaatgatgaagaaattgaattttgtatttattcaagttcagttacaatgctttatagtggtggtaaaaataccgtaagacaggttgatttcactctaaacgaaacccacattagatttacaaaagagttatggagtagatactctgataaagttttagataaacacttagcgttgatagatgattggctacttggaattagtactcctaatagtgataaaactactctcgcttgctttgtttaa

SEQ ID NO: 59 - protein, 575 aa, Artificial
  Amino acid sequence of a TIC7110/TIC6280 fusion toxin protein, TIC7110-TIC6280F3,  wherein a flexible linker peptide sequence (Linker 2) is inserted between the two toxin protein amino acid sequences.
MTNLDLKMESWLALNDISLHQNLEPVAIKLAPSDQTVVSQGIFVGSQLSEARIADNQVQQALQNFGRYSSAVKEAAKVAPTTGLTTILDIARIVSNFNPALPNDKNNVPAYEKYVSKILQNPLIHLLNSSLKSFKRRTSDWNEVIDQIANLYNGISAVDKGKIVESLKALANSASSSSSEKQTEKLFTQSTINCEENIDIYIYSSSVTMEEHNGKHNVKQVEFEIQETQLRFTKELWSLYSDAVLAKHLALMDDWLNGIDTKADNRLSTLTCLVGSGTHQSGKTSGSMSNQDLQMESWLTLNDVSLHQNIQTPLSFDLTSSLQDAAPVQDTISGGLIIGNTQNEAIDANNNVKNALQTYGRFSNEVKESAQVSPIVGLTTILDIARIVSNYNPALPTDQENDETKKARVIAYNQYITKVLQNPLMHLKSNYEKKYTKRTSNWKTAIDEISNLYDGITEKDKEKIKNSLQALAEAASSRSNQANTENIFAQNVIVCNDEEIEFCIYSSSVTMLYSGGKNTVRQVDFTLNETHIRFTKELWSRYSDKVLDKHLALIDDWLLGISTPNSDKTTLACFV

SEQ ID NO: 60 - DNA, 1689 bp, Artificial
  Synthetic sequence encoding a TIC7111/TIC6282 fusion toxin protein, TIC7111-TIC6282F1, wherein the two toxin protein encoding sequences are contiguous and in frame.
atgacaaatcttgacttaaaaatggaaagctggttagcactaaatgatatttctctgcatcaaaatttagagcctgttgctattaaacttgcaccatcagatcaaacagttgtcagtcaaggaatctttgttgggagtcagctgtcggaggctagaatcgctgacaatcaagttcagcaagcacttcaaaactttggacgctatagttctgcagtaaaagaagctgctaaagtagctccaacaactggattaacaactattcttgacattgctagaattgtctctaattttaatccagcattaccaaacgataaaaataatgttcctgcttatgaaaaatatgtgtcaaaaattttacaaaacccacttatccatttattaaatagcagtctaaaatcctttaaacgtaggacttccgattggaatgaagtaattgaccaaatcgccaatttatataatggcatttcggcagttgataaaggaaaaatcgtagaaagcttaaaagcattagcaaattccgcctcttcttctagctcagaaaaacaaactgaaaaactatttactcaaagcacgattaactgtgaggaaaatattgatatttatatttactctagctctgttacaatggaggagcacaatgggaagcataatgtaaagcaagttgaatttgaaatacaagaaacacaattaagatttacaaaagaattgtggagtttatactcagatgctgtgttagcaaaacatctagctttaatggatgattggctcaatggcattgatacaaaagctgacaatcgtttatccactcttacatgcttagttatgtcaaatcaagatttacagatggaaagctggttaacagtaaatgatgtttcccttcatcaaaatattcaaacaccactttctttcgaccttacatcctctttacaagatgctgcacctgtccaagatactataagtggaggtttaattattggtaacacacaaaacgaagctatcgatgccaataataatgtaaaaaatgcactgcaaacatacggtcgttttagtaatgaggtcaaagaatctgctcaagtaagtccgattgttggattaacaactatacttgatattgcaagaatagtttccaattacaacccggctttgcccactgatcaagaaaatgatgaaactaaaaaagcaagagttattgcatacaaccaatatattacgaaggtgttgcaaaatcctttaatgcacttaaaaagcaactatgaaaaaaaatacacaaaacgaacttctaactggaagacagctattgaggaaatcagtaatttatatgatggcatcacagaaaaagataaagagaaaattaaaaatagtttacaagctttagcagaagctgcctcttcaagatcaaatcaagccaatacagaaaatatatttgctcaaaatgttattgtgtgcaatgatgaagaaattgaattttgtatttattcaagttcagttacaatgctttatagtggtggtaaaaataccgtaagacaggttgatttcactctaaacgaaacccacattagatttacaaaagagttatggagtagatactctgataaagttttagataaacacttagcgttgatagatgattggctacttggaattagtactcctaatagtgataaaactactctcgcttgctttgtttaa

SEQ ID NO: 61 - protein, 562 aa, Artificial
  Amino acid sequence of a TIC7111/TIC6282 fusion toxin protein.
MTNLDLKMESWLALNDISLHQNLEPVAIKLAPSDQTVVSQGIFVGSQLSEARIADNQVQQALQNFGRYSSAVKEAAKVAPTTGLTTILDIARIVSNFNPALPNDKNNVPAYEKYVSKILQNPLIHLLNSSLKSFKRRTSDWNEVIDQIANLYNGISAVDKGKIVESLKALANSASSSSSEKQTEKLFTQSTINCEENIDIYIYSSSVTMEEHNGKHNVKQVEFEIQETQLRFTKELWSLYSDAVLAKHLALMDDWLNGIDTKADNRLSTLTCLVMSNQDLQMESWLTVNDVSLHQNIQTPLSFDLTSSLQDAAPVQDTISGGLIIGNTQNEAIDANNNVKNALQTYGRFSNEVKESAQVSPIVGLTTILDIARIVSNYNPALPTDQENDETKKARVIAYNQYITKVLQNPLMHLKSNYEKKYTKRTSNWKTAIEEISNLYDGITEKDKEKIKNSLQALAEAASSRSNQANTENIFAQNVIVCNDEEIEFCIYSSSVTMLYSGGKNTVRQVDFTLNETHIRFTKELWSRYSDKVLDKHLALIDDWLLGISTPNSDKTTLACFV

SEQ ID NO: 62 - DNA, 1707 bp, Artificial
  Synthetic sequence encoding a TIC7111/TIC6282 fusion toxin protein, TIC7111-TIC6282F2, wherein a cleavable linker sequence (Linker 1) is operably linked and in frame between the two toxin protein encoding sequences.
atgacaaatcttgacttaaaaatggaaagctggttagcactaaatgatatttctctgcatcaaaatttagagcctgttgctattaaacttgcaccatcagatcaaacagttgtcagtcaaggaatctttgttgggagtcagctgtcggaggctagaatcgctgacaatcaagttcagcaagcacttcaaaactttggacgctatagttctgcagtaaaagaagctgctaaagtagctccaacaactggattaacaactattcttgacattgctagaattgtctctaattttaatccagcattaccaaacgataaaaataatgttcctgcttatgaaaaatatgtgtcaaaaattttacaaaacccacttatccatttattaaatagcagtctaaaatcctttaaacgtaggacttccgattggaatgaagtaattgaccaaatcgccaatttatataatggcatttcggcagttgataaaggaaaaatcgtagaaagcttaaaagcattagcaaattccgcctcttcttctagctcagaaaaacaaactgaaaaactatttactcaaagcacgattaactgtgaggaaaatattgatatttatatttactctagctctgttacaatggaggagcacaatgggaagcataatgtaaagcaagttgaatttgaaatacaagaaacacaattaagatttacaaaagaattgtggagtttatactcagatgctgtgttagcaaaacatctagctttaatggatgattggctcaatggcattgatacaaaagctgacaatcgtttatccactcttacatgcttagttggtagtggcggtgcttcaatgtcaaatcaagatttacagatggaaagctggttaacagtaaatgatgtttcccttcatcaaaatattcaaacaccactttctttcgaccttacatcctctttacaagatgctgcacctgtccaagatactataagtggaggtttaattattggtaacacacaaaacgaagctatcgatgccaataataatgtaaaaaatgcactgcaaacatacggtcgttttagtaatgaggtcaaagaatctgctcaagtaagtccgattgttggattaacaactatacttgatattgcaagaatagtttccaattacaacccggctttgcccactgatcaagaaaatgatgaaactaaaaaagcaagagttattgcatacaaccaatatattacgaaggtgttgcaaaatcctttaatgcacttaaaaagcaactatgaaaaaaaatacacaaaacgaacttctaactggaagacagctattgaggaaatcagtaatttatatgatggcatcacagaaaaagataaagagaaaattaaaaatagtttacaagctttagcagaagctgcctcttcaagatcaaatcaagccaatacagaaaatatatttgctcaaaatgttattgtgtgcaatgatgaagaaattgaattttgtatttattcaagttcagttacaatgctttatagtggtggtaaaaataccgtaagacaggttgatttcactctaaacgaaacccacattagatttacaaaagagttatggagtagatactctgataaagttttagataaacacttagcgttgatagatgattggctacttggaattagtactcctaatagtgataaaactactctcgcttgctttgtttaa

SEQ ID NO: 63 - protein, 568 aa, Artificial
  Amino acid sequence of a TIC7111/TIC6282 fusion toxin protein, TIC7111-TIC6282F2,  wherein a cleavable linker peptide sequence (Linker 1) is inserted between the two toxin protein amino acid sequences.
MTNLDLKMESWLALNDISLHQNLEPVAIKLAPSDQTVVSQGIFVGSQLSEARIADNQVQQALQNFGRYSSAVKEAAKVAPTTGLTTILDIARIVSNFNPALPNDKNNVPAYEKYVSKILQNPLIHLLNSSLKSFKRRTSDWNEVIDQIANLYNGISAVDKGKIVESLKALANSASSSSSEKQTEKLFTQSTINCEENIDIYIYSSSVTMEEHNGKHNVKQVEFEIQETQLRFTKELWSLYSDAVLAKHLALMDDWLNGIDTKADNRLSTLTCLVGSGGASMSNQDLQMESWLTVNDVSLHQNIQTPLSFDLTSSLQDAAPVQDTISGGLIIGNTQNEAIDANNNVKNALQTYGRFSNEVKESAQVSPIVGLTTILDIARIVSNYNPALPTDQENDETKKARVIAYNQYITKVLQNPLMHLKSNYEKKYTKRTSNWKTAIEEISNLYDGITEKDKEKIKNSLQALAEAASSRSNQANTENIFAQNVIVCNDEEIEFCIYSSSVTMLYSGGKNTVRQVDFTLNETHIRFTKELWSRYSDKVLDKHLALIDDWLLGISTPNSDKTTLACFV

SEQ ID NO: 64 - DNA, 1728 bp, Artificial
  Synthetic sequence encoding a TIC7111/TIC6282 fusion toxin protein, TIC7111-TIC6282F3, wherein a flexible linker sequence (Linker 2) is operably linked and in frame between the two toxin protein encoding sequences.
atgacaaatcttgacttaaaaatggaaagctggttagcactaaatgatatttctctgcatcaaaatttagagcctgttgctattaaacttgcaccatcagatcaaacagttgtcagtcaaggaatctttgttgggagtcagctgtcggaggctagaatcgctgacaatcaagttcagcaagcacttcaaaactttggacgctatagttctgcagtaaaagaagctgctaaagtagctccaacaactggattaacaactattcttgacattgctagaattgtctctaattttaatccagcattaccaaacgataaaaataatgttcctgcttatgaaaaatatgtgtcaaaaattttacaaaacccacttatccatttattaaatagcagtctaaaatcctttaaacgtaggacttccgattggaatgaagtaattgaccaaatcgccaatttatataatggcatttcggcagttgataaaggaaaaatcgtagaaagcttaaaagcattagcaaattccgcctcttcttctagctcagaaaaacaaactgaaaaactatttactcaaagcacgattaactgtgaggaaaatattgatatttatatttactctagctctgttacaatggaggagcacaatgggaagcataatgtaaagcaagttgaatttgaaatacaagaaacacaattaagatttacaaaagaattgtggagtttatactcagatgctgtgttagcaaaacatctagctttaatggatgattggctcaatggcattgatacaaaagctgacaatcgtttatccactcttacatgcttagttggaagcggaacacatcaatctggtaagacatcgggatctatgtcaaatcaagatttacagatggaaagctggttaacagtaaatgatgtttcccttcatcaaaatattcaaacaccactttctttcgaccttacatcctctttacaagatgctgcacctgtccaagatactataagtggaggtttaattattggtaacacacaaaacgaagctatcgatgccaataataatgtaaaaaatgcactgcaaacatacggtcgttttagtaatgaggtcaaagaatctgctcaagtaagtccgattgttggattaacaactatacttgatattgcaagaatagtttccaattacaacccggctttgcccactgatcaagaaaatgatgaaactaaaaaagcaagagttattgcatacaaccaatatattacgaaggtgttgcaaaatcctttaatgcacttaaaaagcaactatgaaaaaaaatacacaaaacgaacttctaactggaagacagctattgaggaaatcagtaatttatatgatggcatcacagaaaaagataaagagaaaattaaaaatagtttacaagctttagcagaagctgcctcttcaagatcaaatcaagccaatacagaaaatatatttgctcaaaatgttattgtgtgcaatgatgaagaaattgaattttgtatttattcaagttcagttacaatgctttatagtggtggtaaaaataccgtaagacaggttgatttcactctaaacgaaacccacattagatttacaaaagagttatggagtagatactctgataaagttttagataaacacttagcgttgatagatgattggctacttggaattagtactcctaatagtgataaaactactctcgcttgctttgtttaa

SEQ ID NO: 65 - protein, 575 aa, Artificial
  Amino acid sequence of a TIC7111/TIC6282 fusion toxin protein, TIC7111-TIC6282F3,  wherein a flexible linker peptide sequence (Linker 2) is inserted between the two toxin protein amino acid sequences.
MTNLDLKMESWLALNDISLHQNLEPVAIKLAPSDQTVVSQGIFVGSQLSEARIADNQVQQALQNFGRYSSAVKEAAKVAPTTGLTTILDIARIVSNFNPALPNDKNNVPAYEKYVSKILQNPLIHLLNSSLKSFKRRTSDWNEVIDQIANLYNGISAVDKGKIVESLKALANSASSSSSEKQTEKLFTQSTINCEENIDIYIYSSSVTMEEHNGKHNVKQVEFEIQETQLRFTKELWSLYSDAVLAKHLALMDDWLNGIDTKADNRLSTLTCLVGSGTHQSGKTSGSMSNQDLQMESWLTVNDVSLHQNIQTPLSFDLTSSLQDAAPVQDTISGGLIIGNTQNEAIDANNNVKNALQTYGRFSNEVKESAQVSPIVGLTTILDIARIVSNYNPALPTDQENDETKKARVIAYNQYITKVLQNPLMHLKSNYEKKYTKRTSNWKTAIEEISNLYDGITEKDKEKIKNSLQALAEAASSRSNQANTENIFAQNVIVCNDEEIEFCIYSSSVTMLYSGGKNTVRQVDFTLNETHIRFTKELWSRYSDKVLDKHLALIDDWLLGISTPNSDKTTLACFV

SEQ ID NO: 66 - DNA, 1689 bp, Artificial
  Synthetic sequence encoding a TIC7109/TIC6281 fusion toxin protein, TIC7109-TIC6281F1, wherein the two toxin protein encoding sequences are contiguous and in frame.
atgacaaatcttgacttaaaaatggaaagctggttagcactaaatgatatttctctgcatcaaaatttagagcctgttgctattaaacttgcaccatcagatcaaacagttgtcagtcaaggaatctttgttgggagtcagctgtcggaggctagaatcgctgacaatcaagttcagcaagcacttcaaaactttggacgctatagttctgcagtaaaagaagctgctaaagtagctccaacaactggattaacaactattcttgatattgctagaattgtttctaattttaatccagcattaccaaacgataaaaataatgttcctgcttatgaaaaatatgtgtcaaaaattttacaaaacccacttatccatttattaaatagcagtctaaaatcctttaaacgtaggacttccgattggaatgaagtaattgaccaaatcgccaatttatataatggcatttcggcagttgataaaggaaaaatcgtagaaagcttaaaagcattagcaaattccgcctcttcttctagctcagaaaaacaaactgaaaaactatttactcaaagcacgattaactgtgaggaaaatattgatatttatatttactctagctctgttacaatggaggagcacaatgggaagcataatgtaaagcaagttgaatttgaaatacaagaaacacaattaagatttacaaaagaattgtggagtttatactcagatgctgtgttagcaaaacatctagctttaatggatgattggctcaatggcattgatacaaaagctgacaatcgtttatccactcttacatgcttagttatgtcaaatcaagatttacagatggaaagctggttaacattaaatgatgtttcccttcatcaaaatattcaaacaccactttctttcgaccttacttcctctttacaagatgctgcacctgtccaagatactataagtggaggtttaattattggtaacacacaaaacgaagctatcgatgccagtaataatgtaaaaaatgcactgcaaacatacggtcgttttagtaatgaggtcaaagaatctgctcaagtaagtccgattgttggattaacaactatacttgatattgcaagaatagtttccaattacaacccggctttgcccactgatcaagaaaatgatgaaactaaaaaagcaagagttattgcatacaaccaatatattacgaaggtgttgcaaaatcctttaatgcacttaaaaagcaactatgaaaaaaaatacacaaaacgaacttctaactggaagacagctattgatgaaatcagtaatttatatgatggcatcacagaaaaagataaagagaaaattaaaaatagtttacaagctttagcagaagctgcttcttcaagatcaaatcaagccaatacagaaaatatatttgctcaaaatgttattgtgtgcaataatgaagaaattgaattttgtatttattcaagttcagttacaatgctttatagtggtggtaaaaataccgtaagacaggttgatttcactctaaacgaaacccacattagatttacaaaagagttatggagtagatactctgataaagttttagataaacacttagcgttgatagatgattggctacttggaattagtactcctaatagtgataaaactactctcgcttgctttgtttaa

SEQ ID NO: 67 - protein, 562 aa, Artificial
  Amino acid sequence of a TIC7109/TIC6281 fusion toxin protein, TIC7109-TIC6281F1, wherein the two toxin protein amino acid sequences are contiguous.
MTNLDLKMESWLALNDISLHQNLEPVAIKLAPSDQTVVSQGIFVGSQLSEARIADNQVQQALQNFGRYSSAVKEAAKVAPTTGLTTILDIARIVSNFNPALPNDKNNVPAYEKYVSKILQNPLIHLLNSSLKSFKRRTSDWNEVIDQIANLYNGISAVDKGKIVESLKALANSASSSSSEKQTEKLFTQSTINCEENIDIYIYSSSVTMEEHNGKHNVKQVEFEIQETQLRFTKELWSLYSDAVLAKHLALMDDWLNGIDTKADNRLSTLTCLVMSNQDLQMESWLTLNDVSLHQNIQTPLSFDLTSSLQDAAPVQDTISGGLIIGNTQNEAIDASNNVKNALQTYGRFSNEVKESAQVSPIVGLTTILDIARIVSNYNPALPTDQENDETKKARVIAYNQYITKVLQNPLMHLKSNYEKKYTKRTSNWKTAIDEISNLYDGITEKDKEKIKNSLQALAEAASSRSNQANTENIFAQNVIVCNNEEIEFCIYSSSVTMLYSGGKNTVRQVDFTLNETHIRFTKELWSRYSDKVLDKHLALIDDWLLGISTPNSDKTTLACFV

SEQ ID NO: 68 - DNA, 1707 bp, Artificial
  Synthetic sequence encoding a TIC7109/TIC6281 fusion toxin protein, TIC7109-TIC6281F2, wherein a cleavable linker sequence (Linker 1) is operably linked and in frame between the two toxin protein encoding sequences.
atgacaaatcttgacttaaaaatggaaagctggttagcactaaatgatatttctctgcatcaaaatttagagcctgttgctattaaacttgcaccatcagatcaaacagttgtcagtcaaggaatctttgttgggagtcagctgtcggaggctagaatcgctgacaatcaagttcagcaagcacttcaaaactttggacgctatagttctgcagtaaaagaagctgctaaagtagctccaacaactggattaacaactattcttgatattgctagaattgtttctaattttaatccagcattaccaaacgataaaaataatgttcctgcttatgaaaaatatgtgtcaaaaattttacaaaacccacttatccatttattaaatagcagtctaaaatcctttaaacgtaggacttccgattggaatgaagtaattgaccaaatcgccaatttatataatggcatttcggcagttgataaaggaaaaatcgtagaaagcttaaaagcattagcaaattccgcctcttcttctagctcagaaaaacaaactgaaaaactatttactcaaagcacgattaactgtgaggaaaatattgatatttatatttactctagctctgttacaatggaggagcacaatgggaagcataatgtaaagcaagttgaatttgaaatacaagaaacacaattaagatttacaaaagaattgtggagtttatactcagatgctgtgttagcaaaacatctagctttaatggatgattggctcaatggcattgatacaaaagctgacaatcgtttatccactcttacatgcttagttggtagtggcggtgcttcaatgtcaaatcaagatttacagatggaaagctggttaacattaaatgatgtttcccttcatcaaaatattcaaacaccactttctttcgaccttacttcctctttacaagatgctgcacctgtccaagatactataagtggaggtttaattattggtaacacacaaaacgaagctatcgatgccagtaataatgtaaaaaatgcactgcaaacatacggtcgttttagtaatgaggtcaaagaatctgctcaagtaagtccgattgttggattaacaactatacttgatattgcaagaatagtttccaattacaacccggctttgcccactgatcaagaaaatgatgaaactaaaaaagcaagagttattgcatacaaccaatatattacgaaggtgttgcaaaatcctttaatgcacttaaaaagcaactatgaaaaaaaatacacaaaacgaacttctaactggaagacagctattgatgaaatcagtaatttatatgatggcatcacagaaaaagataaagagaaaattaaaaatagtttacaagctttagcagaagctgcttcttcaagatcaaatcaagccaatacagaaaatatatttgctcaaaatgttattgtgtgcaataatgaagaaattgaattttgtatttattcaagttcagttacaatgctttatagtggtggtaaaaataccgtaagacaggttgatttcactctaaacgaaacccacattagatttacaaaagagttatggagtagatactctgataaagttttagataaacacttagcgttgatagatgattggctacttggaattagtactcctaatagtgataaaactactctcgcttgctttgtttaa

SEQ ID NO: 69 - protein, 568 aa, Artificial
  Amino acid sequence of a TIC7109/TIC6281 fusion toxin protein, TIC7109-TIC6281F2,  wherein a cleavable linker peptide sequence (Linker 1) is inserted between the two toxin protein amino acid sequences.
MTNLDLKMESWLALNDISLHQNLEPVAIKLAPSDQTVVSQGIFVGSQLSEARIADNQVQQALQNFGRYSSAVKEAAKVAPTTGLTTILDIARIVSNFNPALPNDKNNVPAYEKYVSKILQNPLIHLLNSSLKSFKRRTSDWNEVIDQIANLYNGISAVDKGKIVESLKALANSASSSSSEKQTEKLFTQSTINCEENIDIYIYSSSVTMEEHNGKHNVKQVEFEIQETQLRFTKELWSLYSDAVLAKHLALMDDWLNGIDTKADNRLSTLTCLVGSGGASMSNQDLQMESWLTLNDVSLHQNIQTPLSFDLTSSLQDAAPVQDTISGGLIIGNTQNEAIDASNNVKNALQTYGRFSNEVKESAQVSPIVGLTTILDIARIVSNYNPALPTDQENDETKKARVIAYNQYITKVLQNPLMHLKSNYEKKYTKRTSNWKTAIDEISNLYDGITEKDKEKIKNSLQALAEAASSRSNQANTENIFAQNVIVCNNEEIEFCIYSSSVTMLYSGGKNTVRQVDFTLNETHIRFTKELWSRYSDKVLDKHLALIDDWLLGISTPNSDKTTLACFV

SEQ ID NO: 70 - DNA, 1728 bp, Artificial
  Synthetic sequence encoding a TIC7109/TIC6281 fusion toxin protein, TIC7109-TIC6281F3, wherein a flexible linker sequence (Linker 2) is operably linked and in frame between the two toxin protein encoding sequences.
atgacaaatcttgacttaaaaatggaaagctggttagcactaaatgatatttctctgcatcaaaatttagagcctgttgctattaaacttgcaccatcagatcaaacagttgtcagtcaaggaatctttgttgggagtcagctgtcggaggctagaatcgctgacaatcaagttcagcaagcacttcaaaactttggacgctatagttctgcagtaaaagaagctgctaaagtagctccaacaactggattaacaactattcttgatattgctagaattgtttctaattttaatccagcattaccaaacgataaaaataatgttcctgcttatgaaaaatatgtgtcaaaaattttacaaaacccacttatccatttattaaatagcagtctaaaatcctttaaacgtaggacttccgattggaatgaagtaattgaccaaatcgccaatttatataatggcatttcggcagttgataaaggaaaaatcgtagaaagcttaaaagcattagcaaattccgcctcttcttctagctcagaaaaacaaactgaaaaactatttactcaaagcacgattaactgtgaggaaaatattgatatttatatttactctagctctgttacaatggaggagcacaatgggaagcataatgtaaagcaagttgaatttgaaatacaagaaacacaattaagatttacaaaagaattgtggagtttatactcagatgctgtgttagcaaaacatctagctttaatggatgattggctcaatggcattgatacaaaagctgacaatcgtttatccactcttacatgcttagttggaagcggaacacatcaatctggtaagacatcgggatctatgtcaaatcaagatttacagatggaaagctggttaacattaaatgatgtttcccttcatcaaaatattcaaacaccactttctttcgaccttacttcctctttacaagatgctgcacctgtccaagatactataagtggaggtttaattattggtaacacacaaaacgaagctatcgatgccagtaataatgtaaaaaatgcactgcaaacatacggtcgttttagtaatgaggtcaaagaatctgctcaagtaagtccgattgttggattaacaactatacttgatattgcaagaatagtttccaattacaacccggctttgcccactgatcaagaaaatgatgaaactaaaaaagcaagagttattgcatacaaccaatatattacgaaggtgttgcaaaatcctttaatgcacttaaaaagcaactatgaaaaaaaatacacaaaacgaacttctaactggaagacagctattgatgaaatcagtaatttatatgatggcatcacagaaaaagataaagagaaaattaaaaatagtttacaagctttagcagaagctgcttcttcaagatcaaatcaagccaatacagaaaatatatttgctcaaaatgttattgtgtgcaataatgaagaaattgaattttgtatttattcaagttcagttacaatgctttatagtggtggtaaaaataccgtaagacaggttgatttcactctaaacgaaacccacattagatttacaaaagagttatggagtagatactctgataaagttttagataaacacttagcgttgatagatgattggctacttggaattagtactcctaatagtgataaaactactctcgcttgctttgtttaa

SEQ ID NO: 71 - protein, 575 aa, Artificial
  Amino acid sequence of a TIC7109/TIC6281 fusion toxin protein, TIC7109-TIC6281F3,  wherein a flexible linker peptide sequence (Linker 2) is inserted between the two toxin protein amino acid sequences.
MTNLDLKMESWLALNDISLHQNLEPVAIKLAPSDQTVVSQGIFVGSQLSEARIADNQVQQALQNFGRYSSAVKEAAKVAPTTGLTTILDIARIVSNFNPALPNDKNNVPAYEKYVSKILQNPLIHLLNSSLKSFKRRTSDWNEVIDQIANLYNGISAVDKGKIVESLKALANSASSSSSEKQTEKLFTQSTINCEENIDIYIYSSSVTMEEHNGKHNVKQVEFEIQETQLRFTKELWSLYSDAVLAKHLALMDDWLNGIDTKADNRLSTLTCLVGSGTHQSGKTSGSMSNQDLQMESWLTLNDVSLHQNIQTPLSFDLTSSLQDAAPVQDTISGGLIIGNTQNEAIDASNNVKNALQTYGRFSNEVKESAQVSPIVGLTTILDIARIVSNYNPALPTDQENDETKKARVIAYNQYITKVLQNPLMHLKSNYEKKYTKRTSNWKTAIDEISNLYDGITEKDKEKIKNSLQALAEAASSRSNQANTENIFAQNVIVCNNEEIEFCIYSSSVTMLYSGGKNTVRQVDFTLNETHIRFTKELWSRYSDKVLDKHLALIDDWLLGISTPNSDKTTLACFV

SEQ ID NO: 72 - DNA, 18 bp, Artificial
  Synthetic DNA sequence encoding a cleavable linker, Linker 1 that is operably linked and in frame between two toxin coding sequences.
ggtagtggcggtgcttca

SEQ ID NO: 73 - protein, 6 aa, Artificial
  Amino acid sequence of the cleavable linker, Linker 1.
GSGGAS

SEQ ID NO: 74 - DNA, 39 bp, Artificial
  Synthetic DNA sequence encoding a flexible linker, Linker 2 that is operably linked and in frame between two toxin coding sequences.
ggaagcggaacacatcaatctggtaagacatcgggatct

SEQ ID NO: 75 - protein, 13 aa, Artificial
  Amino acid sequence of the flexible linker, Linker 2.
GSGTHQSGKTSGS

SEQ ID NO: 76 - DNA, 1749 bp, Artificial
  Synthetic sequence of an operon, TIC7110-TIC6280operon, comprising the coding sequence of TIC7110 followed by the coding sequence of TIC6280, wherein an operon linker (Operon_Linker) is inserted between the two coding sequences.
atgacaaatcttgacttaaaaatggaaagctggttagcactaaatgatatttctctgcatcaaaatttagagcctgttgctattaaacttgcaccatcagatcaaacagttgtcagtcaaggaatctttgttgggagtcagctgtcggaggctagaatcgctgacaatcaagttcagcaagcacttcaaaactttggacgctatagttctgcagtaaaagaagctgctaaagtagctccaacaactggattaacaactattcttgatattgctagaattgtttctaattttaatccagcattaccaaacgataaaaataatgttcctgcttatgaaaaatatgtgtcaaaaattttacaaaacccacttatccatttattaaatagcagtctaaaatcctttaaacgtaggacttccgattggaatgaagtaattgaccaaatcgccaatttatataatggcatttcggcagttgataaaggaaaaatcgtagaaagcttaaaagcattagcaaattccgcctcttcttctagctcagaaaaacaaactgaaaaactatttactcaaagcacgattaactgtgaggaaaatattgatatttatatttactctagctctgttacaatggaggagcacaatgggaagcataatgtaaagcaagttgaatttgaaatacaagaaactcaattaagatttacaaaagaattgtggagtttatactcagatgctgtgttagcaaaacatctagctttaatggatgattggctcaatggcattgatacaaaagctgacaatcgtttatccactcttacatgcttagtttaacaaaatcaaatagattaattgcaatgaagttttttatatgttttttaaggaggaaataatatgtcaaatcaagatttacagatggaaagctggttaacattaaatgatgtttcccttcatcaaaatattcaaacaccactttctttcgaccttacttcctctttacaagatgctgcacctgtccaagatactataagtggaggtttaattattggtaacacacaaaacgaagctatcgatgccaataataatgtaaaaaatgcactgcaaacatacggtcgttttagtaatgaggtcaaagaatctgctcaagtaagtccgattgttggattaacaactatacttgatattgcaagaatagtttccaattacaacccggctttgcccactgatcaagaaaatgatgaaactaaaaaagcaagagttattgcatacaaccaatatattacgaaggtgttgcaaaatcctttaatgcacttaaaaagcaactatgaaaaaaaatacacaaaacgaacttctaactggaagacagctattgatgaaatcagtaatttatatgatggcatcacagaaaaagataaagagaaaattaaaaatagtttacaagctttagcagaagctgcttcttcaagatcaaatcaagccaatacagaaaatatatttgctcaaaatgttattgtgtgcaatgatgaagaaattgaattttgtatttattcaagttcagttacaatgctttatagtggtggtaaaaataccgtaagacaggttgatttcactctaaacgaaacccacattagatttacaaaagagttatggagtagatactctgataaagttttagataaacacttagcgttgatagatgattggctacttggaattagtactcctaatagtgataaaactactctcgcttgctttgtt

SEQ ID NO: 77 - DNA, 1749 bp, Artificial
  Synthetic sequence of an operon, TIC7111-TIC6282operon, comprising the coding sequence of TIC7111 followed by the coding sequence of TIC6282, wherein an operon linker (Operon_Linker) is inserted between the two coding sequences.
atgacaaatcttgacttaaaaatggaaagctggttagcactaaatgatatttctctgcatcaaaatttagagcctgttgctattaaacttgcaccatcagatcaaacagttgtcagtcaaggaatctttgttgggagtcagctgtcggaggctagaatcgctgacaatcaagttcagcaagcacttcaaaactttggacgctatagttctgcagtaaaagaagctgctaaagtagctccaacaactggattaacaactattcttgacattgctagaattgtctctaattttaatccagcattaccaaacgataaaaataatgttcctgcttatgaaaaatatgtgtcaaaaattttacaaaacccacttatccatttattaaatagcagtctaaaatcctttaaacgtaggacttccgattggaatgaagtaattgaccaaatcgccaatttatataatggcatttcggcagttgataaaggaaaaatcgtagaaagcttaaaagcattagcaaattccgcctcttcttctagctcagaaaaacaaactgaaaaactatttactcaaagcacgattaactgtgaggaaaatattgatatttatatttactctagctctgttacaatggaggagcacaatgggaagcataatgtaaagcaagttgaatttgaaatacaagaaacacaattaagatttacaaaagaattgtggagtttatactcagatgctgtgttagcaaaacatctagctttaatggatgattggctcaatggcattgatacaaaagctgacaatcgtttatccactcttacatgcttagtttaacaaaatcaaatagattaattgcaatgaagttttttatatgttttttaaggaggaaataatatgtcaaatcaagatttacagatggaaagctggttaacagtaaatgatgtttcccttcatcaaaatattcaaacaccactttctttcgaccttacatcctctttacaagatgctgcacctgtccaagatactataagtggaggtttaattattggtaacacacaaaacgaagctatcgatgccaataataatgtaaaaaatgcactgcaaacatacggtcgttttagtaatgaggtcaaagaatctgctcaagtaagtccgattgttggattaacaactatacttgatattgcaagaatagtttccaattacaacccggctttgcccactgatcaagaaaatgatgaaactaaaaaagcaagagttattgcatacaaccaatatattacgaaggtgttgcaaaatcctttaatgcacttaaaaagcaactatgaaaaaaaatacacaaaacgaacttctaactggaagacagctattgaggaaatcagtaatttatatgatggcatcacagaaaaagataaagagaaaattaaaaatagtttacaagctttagcagaagctgcctcttcaagatcaaatcaagccaatacagaaaatatatttgctcaaaatgttattgtgtgcaatgatgaagaaattgaattttgtatttattcaagttcagttacaatgctttatagtggtggtaaaaataccgtaagacaggttgatttcactctaaacgaaacccacattagatttacaaaagagttatggagtagatactctgataaagttttagataaacacttagcgttgatagatgattggctacttggaattagtactcctaatagtgataaaactactctcgcttgctttgtt

SEQ ID NO: 78 - DNA, 1749 bp, Artificial
  Synthetic sequence of an operon, TIC7109-TIC6281operon, comprising the coding sequence of TIC7109 followed by the coding sequence of TIC6281, wherein an operon linker (Operon_Linker) is inserted between the two coding sequences.
atgacaaatcttgacttaaaaatggaaagctggttagcactaaatgatatttctctgcatcaaaatttagagcctgttgctattaaacttgcaccatcagatcaaacagttgtcagtcaaggaatctttgttgggagtcagctgtcggaggctagaatcgctgacaatcaagttcagcaagcacttcaaaactttggacgctatagttctgcagtaaaagaagctgctaaagtagctccaacaactggattaacaactattcttgatattgctagaattgtttctaattttaatccagcattaccaaacgataaaaataatgttcctgcttatgaaaaatatgtgtcaaaaattttacaaaacccacttatccatttattaaatagcagtctaaaatcctttaaacgtaggacttccgattggaatgaagtaattgaccaaatcgccaatttatataatggcatttcggcagttgataaaggaaaaatcgtagaaagcttaaaagcattagcaaattccgcctcttcttctagctcagaaaaacaaactgaaaaactatttactcaaagcacgattaactgtgaggaaaatattgatatttatatttactctagctctgttacaatggaggagcacaatgggaagcataatgtaaagcaagttgaatttgaaatacaagaaacacaattaagatttacaaaagaattgtggagtttatactcagatgctgtgttagcaaaacatctagctttaatggatgattggctcaatggcattgatacaaaagctgacaatcgtttatccactcttacatgcttagtttaacaaaatcaaatagattaattgcaatgaagttttttatatgttttttaaggaggaaataatatgtcaaatcaagatttacagatggaaagctggttaacattaaatgatgtttcccttcatcaaaatattcaaacaccactttctttcgaccttacttcctctttacaagatgctgcacctgtccaagatactataagtggaggtttaattattggtaacacacaaaacgaagctatcgatgccagtaataatgtaaaaaatgcactgcaaacatacggtcgttttagtaatgaggtcaaagaatctgctcaagtaagtccgattgttggattaacaactatacttgatattgcaagaatagtttccaattacaacccggctttgcccactgatcaagaaaatgatgaaactaaaaaagcaagagttattgcatacaaccaatatattacgaaggtgttgcaaaatcctttaatgcacttaaaaagcaactatgaaaaaaaatacacaaaacgaacttctaactggaagacagctattgatgaaatcagtaatttatatgatggcatcacagaaaaagataaagagaaaattaaaaatagtttacaagctttagcagaagctgcttcttcaagatcaaatcaagccaatacagaaaatatatttgctcaaaatgttattgtgtgcaataatgaagaaattgaattttgtatttattcaagttcagttacaatgctttatagtggtggtaaaaataccgtaagacaggttgatttcactctaaacgaaacccacattagatttacaaaagagttatggagtagatactctgataaagttttagataaacacttagcgttgatagatgattggctacttggaattagtactcctaatagtgataaaactactctcgcttgctttgtt

SEQ ID NO: 79 - DNA, 40 bp, Artificial
  Synthetic sequence of a linker, Operon_Linker which comprises at the 5' end a stop codon to terminate translation of a first toxin gene and is inserted between two toxin protein coding sequences to permit expression of both toxin proteins in the bacterial host
taacaaaatcaaatagattaattgcaatgaagttttttat

SEQ ID NO: 80 - DNA, 885 bp, Artificial
  Nucleic acid sequence obtained from a metagenome designated MTG000070, encoding a TIC8808 pesticidal protein with a Histidine tag operably linked to the 3' end, TIC8808-His.
atgtcaaatcaagatttacagatggaaagctggttaacagtaaatgatgtttcacttcatcaaaatattcaaacaccactttctttcgaccatactacatctctacaagatacaacacctgtccaagacactataagtggaggtttaattattggtcacaaacaaaatgaagctattgatgccaataataatgtaaaaaatgcattacaaacgtatgaccgttttagtaatgaggtcaaagaatctgcccaaataagtccaattgttggattaacaactatacttgatatcgcaagaatagtttccaattacaatcctgctttgcccactgaccaagaaaataatgaaactaaaaaagcaaaagttgctgcatacaaccaatatattacgaaggtgctgcaaaatcctttaatgcacttaaaaagcaactatgaaaaaaaatacacgaaaataacttctaactggaagacagctattgatgaaattagtaatttatatgatgggatcacagaaaaagataaagagaaaattaaaactagtttacacgctttagcagaagctgcctcttcaagatcaaataaagccaatacagaaaatatatttgctcaaaatgtcatagtgtgcaatgatgaagaaattgaattttgcatttattcaagttcagttacaatgctttatagtgatggtaaaaataccgtgagacaggttgattttacactaaacgaaacccacattagatttacaaaagaattatggagtagatattctgatattgttttagctaaacacttagcgttgttcgatgattggctacttggtattagtacacctaatagtgataaaactactcttgcttgctttgctcaccatcatcaccatcactag

SEQ ID NO: 81 - protein, 295 aa, Artificial
  The amino acid sequence of the TIC8808-His protein.
MSNQDLQMESWLTVNDVSLHQNIQTPLSFDHTTSLQDTTPVQDTISGGLIIGHKQNEAIDANNNVKNALQTYDRFSNEVKESAQISPIVGLTTILDIARIVSNYNPALPTDQENNETKKAKVAAYNQYITKVLQNPLMHLKSNYEKKYTKITSNWKTAIDEISNLYDGITEKDKEKIKTSLHALAEAASSRSNKANTENIFAQNVIVCNDEEIEFCIYSSSVTMLYSDGKNTVRQVDFTLNETHIRFTKELWSRYSDIVLAKHLALFDDWLLGISTPNSDKTTLACFAHHHHHHH

SEQ ID NO: 82 - DNA, 930 bp, Artificial
  Nucleic acid sequence obtained from a metagenome designated MTG000415, encoding a TIC9480 pesticidal protein with a Histidine tag operably linked to the 3' end, TIC9480-His.
atgtcaaatcaagatttacagatggaaagctggttaacagtaaatgatgtttcacttcatcaaaatattcaaacaccactttctttcgaccatactacatctctacaagatacaacacctgtccaagacactataagtggaggtttaattattggtcacaaacaaaatgaagctattgatgccaataataatgtaaaaaatgcattacaaacgtatgaccgttttagtaatgaggtcaaagaatctgcccaaataagtccaattgttggattaacaactatacttgatatcgcaagaatagtttccaattacaatcctgctttgcccactgaccaagaaaataatgaaactaaaaaagcaaaagttgctgcatacaaccaatatattacgaaggtgctgcaaaatcctttaatgcacttaaaaagcaactatgaaaaaaaatacacgaaaataacttctaactggaagacagctattgatgaaattagtaatttatatgatgggatcacagaaaaagataaagagaaaattaaaactagtttacacgctttagcagaagctgcctcttcaagatcaaataaagccaatacagaaaatatatttgctcaaaatgtcatagtgtgcaatgatgaagaaattgaattttgcatttattcaagttcagttacaatgctttatagtgatggtaaaaataccgtgagacaggttgattttacactaaacgaaacccacattagatttacaaaagaattatggagtagatattctgatattgttttagctaagcgttgttcgatgattggctacttggtattagtacacctaatagtgataaaactactcttgcttgctttgcttaaaatatctatcaaaaggaaactagataactttttgtttccttttgatcttcaccatcatcaccatcactag

SEQ ID NO: 83 - protein, 310 aa, Artificial
  The amino acid sequence of the TIC9480-His protein.
MSNQDLQMESWLTVNDVSLHQNIQTPLSFDHTTSLQDTTPVQDTISGGLIIGHKQNEAIDANNNVKNALQTYDRFSNEVKESAQISPIVGLTTILDIARIVSNYNPALPTDQENNETKKAKVAAYNQYITKVLQNPLMHLKSNYEKKYTKITSNWKTAIDEISNLYDGITEKDKEKIKTSLHALAEAASSRSNKANTENIFAQNVIVCNDEEIEFCIYSSSVTMLYSDGKNTVRQVDFTLNETHIRFTKELWSRYSDIVLAKRCSMIGYLVLVHLIVIKLLLLALLKISIKRKLDNFLFPFDLHHHHHHH

SEQ ID NO: 84 - DNA, 930 bp, Artificial
  Nucleic acid sequence obtained from a metagenome designated MTG000199, encoding a TIC9257 pesticidal protein with a Histidine tag operably linked to the 3' end, TIC9257-His.
atgtcaaatcaagatttacagatggaaagctggttaacagtaaatgatgtttcacttcatcaaaatattcaaacaccactttctttcgaccatactacatctctacaagatacaacacctgtccaagacactataagtggaggtttaattattggtcacaaacaaaatgaagctattgatgccaataataatgtaaaaaatgcattacaaacgtatgaccgttttagtaatgaggtcaaagaatctgcccaaataagtccaattgttggattaacaactatacttgatatcgcaagaatagtttccaattacaatcctgctttgcccactgaccaagaaaataatgaaactaaaaaagcaaaagttgctgcatacaaccaatatattacgaaggtgctgcaaaatcctttaatgcacttaaaaagcaactatgaaaaaaaatacacgaaaataacttctaactggaagacagctattgatgaaattagtaatttatatgatgggatcacagaaaaagataaagagaaaattaaaactagtttacacgctttagcagaagctgcctcttcaagatcaaataaagccaatacagaaaatatatttgctcaaaatgtcatagtgtgcaatgatgaagaaattgaattttgcatttattcaagttcagttacaatgctttatagtgatggtaaaaataccgtgagacaggttgattttacactaaacgaaacccacattagatttacaaaagaattatggagtagatattctgatattgttttagctaagcgttgttcgatgattggctacttggtattagtacacctaatagtgataaaactactcttgcttgctttgcttaaaatatctatcaaaaggaaactagaaaactttttgtttccttttgatcttcaccatcatcaccatcactag

SEQ ID NO: 85 - protein, 310 aa, Artificial
  The amino acid sequence of the TIC9257-His protein.
MSNQDLQMESWLTVNDVSLHQNIQTPLSFDHTTSLQDTTPVQDTISGGLIIGHKQNEAIDANNNVKNALQTYDRFSNEVKESAQISPIVGLTTILDIARIVSNYNPALPTDQENNETKKAKVAAYNQYITKVLQNPLMHLKSNYEKKYTKITSNWKTAIDEISNLYDGITEKDKEKIKTSLHALAEAASSRSNKANTENIFAQNVIVCNDEEIEFCIYSSSVTMLYSDGKNTVRQVDFTLNETHIRFTKELWSRYSDIVLAKRCSMIGYLVLVHLIVIKLLLLALLKISIKRKLENFLFPFDLHHHHHHH

SEQ ID NO: 86 - DNA, 849 bp, Artificial
  Nucleic acid sequence obtained from a metagenome designated MTG000120, encoding a TIC9258 pesticidal protein with a Histidine tag operably linked to the 3' end, TIC9258-His.
atgacaaatcttgacttaaaaatggaaagctggttagcactaaatgatatttctctacatcaaaatttagagcctgttgctattaaacttgcaacatcagatcaaacagttgtcagtcaaggtatctttgttgggaatcagctgtcagaggctagaattgctgacaatcaagttcagcaggcacttcaaagctttggacgctatagtactgctgtaaaagaagctgctaaagtagctccaacaactggattaacaactatccttgacatttctagaattgtttctaatttcaacccagcattaccaaacgataaaaataatgtacctgcctatgaaaaatatgtttcaaaaatattacaaaacccacttatccatttattaaatagcagtgtaaaatccttcaaacgtacgacttccgattggaatgaagcaattgaccaaattgccaatttatataatggcatttcggcagctgacaaaggaaaaattgtagaaagcttaaaagcattagcaaaatccgcctcttcttctagctctgaaaaacaaacggaaaaactatttactcaaagtacgattaactgtgaggaaaatatagatatttatatttactctagctctgtcacaatggaggagcacaacggtaagcacaatgtaaagcaggttgaatttgaaatacaagaaacacaattaagatttacaaaagaattgtggagtgtatactctgatgctgtgttagctaaacatctagctctaatggatgattggctaaatggtattgatacaaaagcagacaatcgtttatccactcttacttgcttagttcaccaccatcacgctcaccatcactga

SEQ ID NO: 87 - protein, 282 aa, Artificial
  The amino acid sequence of the TIC9258-His protein.
MTNLDLKMESWLALNDISLHQNLEPVAIKLATSDQTVVSQGIFVGNQLSEARIADNQVQQALQSFGRYSTAVKEAAKVAPTTGLTTILDISRIVSNFNPALPNDKNNVPAYEKYVSKILQNPLIHLLNSSVKSFKRTTSDWNEAIDQIANLYNGISAADKGKIVESLKALAKSASSSSSEKQTEKLFTQSTINCEENIDIYIYSSSVTMEEHNGKHNVKQVEFEIQETQLRFTKELWSVYSDAVLAKHLALMDDWLNGIDTKADNRLSTLTCLVHHHHAHHH

SEQ ID NO: 88 - DNA, 849 bp, Artificial
  Nucleic acid sequence obtained from a designated MTG000184, encoding a TIC9259 pesticidal protein with a Histidine tag operably linked to the 3' end, TIC9259-His.
atgacaaatcttgacttaaaaatggaaagttggttagcactaaatgatatttctctacatcaaaatttagagcctgttgctattaaactcgcaacatcagatcaaacagttgtcagtcaaggaatctttgtagggaatcagttgtcggaggctagaattgctgacaatcaggttcagcaggcacttcaaagctttggacgctatagtactgctgtaaaagaagctgctaaagtagctccaacaactggtttaacaactatccttgacattgctagcatcgtttctaatttcaatccggcattaccaaacgataaaaataatgtacctgcctatgaaaaatatgtttcaaaaatattacaaaacccacttatccatttattaaatagcagtgtaaaatccttcaaacgtacgacttctgattggaatgaagcaattgaccaaattgccaatttatataatggcatttcggcagctgacaaaggaaaaattgtagaaagcttaaaagcattagcaaaatccgcctcctcttctagctctgaaaaacaaacggaaaaactatttactcaaagtacgattaactgtgaggaaaatatagatatttatatttactctagctctgtcacaatggaggagcacaacggtaagcacaatgtaaagcaggttgaatttgaaatacaagaaacacaattaagatttacaaaagaattgtggagtttatactctgatgctgtgttagctaaacatctagctctaatggatgattggctaaatggcattgatacaaaagcagacaatcgtttatccactcttacatgcttagttcaccaccatcacgctcaccatcactga

SEQ ID NO: 89 - protein, 282 aa, Artificial
  The amino acid sequence of the TIC9259-His protein.
MTNLDLKMESWLALNDISLHQNLEPVAIKLATSDQTVVSQGIFVGNQLSEARIADNQVQQALQSFGRYSTAVKEAAKVAPTTGLTTILDIASIVSNFNPALPNDKNNVPAYEKYVSKILQNPLIHLLNSSVKSFKRTTSDWNEAIDQIANLYNGISAADKGKIVESLKALAKSASSSSSEKQTEKLFTQSTINCEENIDIYIYSSSVTMEEHNGKHNVKQVEFEIQETQLRFTKELWSLYSDAVLAKHLALMDDWLNGIDTKADNRLSTLTCLVHHHHAHHH

SEQ ID NO: 90 - DNA, 867 bp, Unknown
  Nucleic acid sequence obtained from a plate-scrape metagenome designated MTG000184, encoding a TIC8808 pesticidal protein.
atgtcaaatcaagatttacagatggaaagctggttaacagtaaatgatgtttcacttcatcaaaatattcaaacaccactttctttcgaccatactacatctctacaagatacaacacctgtccaagacactataagtggaggtttaattattggtcacaaacaaaatgaagctattgatgccaataataatgtaaaaaatgcattacaaacgtatgaccgttttagtaatgaggtcaaagaatctgcccaaataagtccaattgttggattaacaactatacttgatatcgcaagaatagtttccaattacaatcctgctttgcccactgaccaagaaaataatgaaactaaaaaagcaaaagttgctgcatacaaccaatatattacgaaggtgctgcaaaatcctttaatgcacttaaaaagcaactatgaaaaaaaatacacgaaaataacttctaactggaagacagctattgatgaaattagtaatttatatgatgggatcacagaaaaagataaagagaaaattaaaactagtttacacgctttagcagaagctgcctcttcaagatcaaataaagccaatacagaaaatatatttgctcaaaatgtcatagtgtgcaatgatgaagaaattgaattttgcatttattcaagttcagttacaatgctttatagtgatggtaaaaataccgtgagacaggttgattttacactaaacgaaacccacattagatttacaaaagaattatggagtagatattctgatattgttttagctaaacacttagcgttgttcgatgattggctacttggtattagtacacctaatagtgataaaactactcttgcttgctttgcttga

SEQ ID NO: 91 - protein, 288 aa, Unknown
  The amino acid sequence of the TIC8808 protein.
MSNQDLQMESWLTVNDVSLHQNIQTPLSFDHTTSLQDTTPVQDTISGGLIIGHKQNEAIDANNNVKNALQTYDRFSNEVKESAQISPIVGLTTILDIARIVSNYNPALPTDQENNETKKAKVAAYNQYITKVLQNPLMHLKSNYEKKYTKITSNWKTAIDEISNLYDGITEKDKEKIKTSLHALAEAASSRSNKANTENIFAQNVIVCNDEEIEFCIYSSSVTMLYSDGKNTVRQVDFTLNETHIRFTKELWSRYSDIVLAKHLALFDDWLLGISTPNSDKTTLACFA

SEQ ID NO: 92 - DNA, 912 bp, Unknown
  Nucleic acid sequence obtained from a plate-scrape metagenome designated MTG000415, encoding a TIC9480 pesticidal protein.
atgtcaaatcaagatttacagatggaaagctggttaacagtaaatgatgtttcacttcatcaaaatattcaaacaccactttctttcgaccatactacatctctacaagatacaacacctgtccaagacactataagtggaggtttaattattggtcacaaacaaaatgaagctattgatgccaataataatgtaaaaaatgcattacaaacgtatgaccgttttagtaatgaggtcaaagaatctgcccaaataagtccaattgttggattaacaactatacttgatatcgcaagaatagtttccaattacaatcctgctttgcccactgaccaagaaaataatgaaactaaaaaagcaaaagttgctgcatacaaccaatatattacgaaggtgctgcaaaatcctttaatgcacttaaaaagcaactatgaaaaaaaatacacgaaaataacttctaactggaagacagctattgatgaaattagtaatttatatgatgggatcacagaaaaagataaagagaaaattaaaactagtttacacgctttagcagaagctgcctcttcaagatcaaataaagccaatacagaaaatatatttgctcaaaatgtcatagtgtgcaatgatgaagaaattgaattttgcatttattcaagttcagttacaatgctttatagtgatggtaaaaataccgtgagacaggttgattttacactaaacgaaacccacattagatttacaaaagaattatggagtagatattctgatattgttttagctaagcgttgttcgatgattggctacttggtattagtacacctaatagtgataaaactactcttgcttgctttgcttaaaatatctatcaaaaggaaactagataactttttgtttccttttgatctttga

SEQ ID NO: 93 - protein, 303 aa, Unknown
  The amino acid sequence of the TIC9480 protein.
MSNQDLQMESWLTVNDVSLHQNIQTPLSFDHTTSLQDTTPVQDTISGGLIIGHKQNEAIDANNNVKNALQTYDRFSNEVKESAQISPIVGLTTILDIARIVSNYNPALPTDQENNETKKAKVAAYNQYITKVLQNPLMHLKSNYEKKYTKITSNWKTAIDEISNLYDGITEKDKEKIKTSLHALAEAASSRSNKANTENIFAQNVIVCNDEEIEFCIYSSSVTMLYSDGKNTVRQVDFTLNETHIRFTKELWSRYSDIVLAKRCSMIGYLVLVHLIVIKLLLLALLKISIKRKLDNFLFPFDL

SEQ ID NO: 94 - DNA, 912 bp, Unknown
  Nucleic acid sequence obtained from a plate-scrape metagenome designated MTG000199, encoding a TIC9257 pesticidal protein.
atgtcaaatcaagatttacagatggaaagctggttaacagtaaatgatgtttcacttcatcaaaatattcaaacaccactttctttcgaccatactacatctctacaagatacaacacctgtccaagacactataagtggaggtttaattattggtcacaaacaaaatgaagctattgatgccaataataatgtaaaaaatgcattacaaacgtatgaccgttttagtaatgaggtcaaagaatctgcccaaataagtccaattgttggattaacaactatacttgatatcgcaagaatagtttccaattacaatcctgctttgcccactgaccaagaaaataatgaaactaaaaaagcaaaagttgctgcatacaaccaatatattacgaaggtgctgcaaaatcctttaatgcacttaaaaagcaactatgaaaaaaaatacacgaaaataacttctaactggaagacagctattgatgaaattagtaatttatatgatgggatcacagaaaaagataaagagaaaattaaaactagtttacacgctttagcagaagctgcctcttcaagatcaaataaagccaatacagaaaatatatttgctcaaaatgtcatagtgtgcaatgatgaagaaattgaattttgcatttattcaagttcagttacaatgctttatagtgatggtaaaaataccgtgagacaggttgattttacactaaacgaaacccacattagatttacaaaagaattatggagtagatattctgatattgttttagctaagcgttgttcgatgattggctacttggtattagtacacctaatagtgataaaactactcttgcttgctttgcttaaaatatctatcaaaaggaaactagaaaactttttgtttccttttgatctttga

SEQ ID NO: 95 - protein, 303 aa, Unknown
  The amino acid sequence of the TIC9257 protein.
MSNQDLQMESWLTVNDVSLHQNIQTPLSFDHTTSLQDTTPVQDTISGGLIIGHKQNEAIDANNNVKNALQTYDRFSNEVKESAQISPIVGLTTILDIARIVSNYNPALPTDQENNETKKAKVAAYNQYITKVLQNPLMHLKSNYEKKYTKITSNWKTAIDEISNLYDGITEKDKEKIKTSLHALAEAASSRSNKANTENIFAQNVIVCNDEEIEFCIYSSSVTMLYSDGKNTVRQVDFTLNETHIRFTKELWSRYSDIVLAKRCSMIGYLVLVHLIVIKLLLLALLKISIKRKLENFLFPFDL

SEQ ID NO: 96 - DNA, 825 bp, Unknown
  Nucleic acid sequence obtained from a plate-scrape metagenome designated MTG000120, encoding a TIC9258 pesticidal protein.
atgacaaatcttgacttaaaaatggaaagctggttagcactaaatgatatttctctacatcaaaatttagagcctgttgctattaaacttgcaacatcagatcaaacagttgtcagtcaaggtatctttgttgggaatcagctgtcagaggctagaattgctgacaatcaagttcagcaggcacttcaaagctttggacgctatagtactgctgtaaaagaagctgctaaagtagctccaacaactggattaacaactatccttgacatttctagaattgtttctaatttcaacccagcattaccaaacgataaaaataatgtacctgcctatgaaaaatatgtttcaaaaatattacaaaacccacttatccatttattaaatagcagtgtaaaatccttcaaacgtacgacttccgattggaatgaagcaattgaccaaattgccaatttatataatggcatttcggcagctgacaaaggaaaaattgtagaaagcttaaaagcattagcaaaatccgcctcttcttctagctctgaaaaacaaacggaaaaactatttactcaaagtacgattaactgtgaggaaaatatagatatttatatttactctagctctgtcacaatggaggagcacaacggtaagcacaatgtaaagcaggttgaatttgaaatacaagaaacacaattaagatttacaaaagaattgtggagtgtatactctgatgctgtgttagctaaacatctagctctaatggatgattggctaaatggtattgatacaaaagcagacaatcgtttatccactcttacttgcttagtttaa

SEQ ID NO: 97 - protein, 274 aa, Unknown
  The amino acid sequence of the TIC9258 protein.
MTNLDLKMESWLALNDISLHQNLEPVAIKLATSDQTVVSQGIFVGNQLSEARIADNQVQQALQSFGRYSTAVKEAAKVAPTTGLTTILDISRIVSNFNPALPNDKNNVPAYEKYVSKILQNPLIHLLNSSVKSFKRTTSDWNEAIDQIANLYNGISAADKGKIVESLKALAKSASSSSSEKQTEKLFTQSTINCEENIDIYIYSSSVTMEEHNGKHNVKQVEFEIQETQLRFTKELWSVYSDAVLAKHLALMDDWLNGIDTKADNRLSTLTCLV

SEQ ID NO: 98 - DNA, 825 bp, Unknown
  Nucleic acid sequence obtained from a plate-scrape metagenome designated MTG000184, encoding a TIC9259 pesticidal protein.
atgacaaatcttgacttaaaaatggaaagttggttagcactaaatgatatttctctacatcaaaatttagagcctgttgctattaaactcgcaacatcagatcaaacagttgtcagtcaaggaatctttgtagggaatcagttgtcggaggctagaattgctgacaatcaggttcagcaggcacttcaaagctttggacgctatagtactgctgtaaaagaagctgctaaagtagctccaacaactggtttaacaactatccttgacattgctagcatcgtttctaatttcaatccggcattaccaaacgataaaaataatgtacctgcctatgaaaaatatgtttcaaaaatattacaaaacccacttatccatttattaaatagcagtgtaaaatccttcaaacgtacgacttctgattggaatgaagcaattgaccaaattgccaatttatataatggcatttcggcagctgacaaaggaaaaattgtagaaagcttaaaagcattagcaaaatccgcctcctcttctagctctgaaaaacaaacggaaaaactatttactcaaagtacgattaactgtgaggaaaatatagatatttatatttactctagctctgtcacaatggaggagcacaacggtaagcacaatgtaaagcaggttgaatttgaaatacaagaaacacaattaagatttacaaaagaattgtggagtttatactctgatgctgtgttagctaaacatctagctctaatggatgattggctaaatggcattgatacaaaagcagacaatcgtttatccactcttacatgcttagtttaa

SEQ ID NO: 99 - protein, 274 aa, Unknown
  The amino acid sequence of the TIC9259 protein.
MTNLDLKMESWLALNDISLHQNLEPVAIKLATSDQTVVSQGIFVGNQLSEARIADNQVQQALQSFGRYSTAVKEAAKVAPTTGLTTILDIASIVSNFNPALPNDKNNVPAYEKYVSKILQNPLIHLLNSSVKSFKRTTSDWNEAIDQIANLYNGISAADKGKIVESLKALAKSASSSSSEKQTEKLFTQSTINCEENIDIYIYSSSVTMEEHNGKHNVKQVEFEIQETQLRFTKELWSLYSDAVLAKHLALMDDWLNGIDTKADNRLSTLTCLV